European Patent Specification EP 4 669 337 B1, published June 24, 2026. Title: AGENTS USEFUL FOR THE PREVENTION OR TREATMENT OF ALLERGIC & INFLAMMATORY DISORDERS. Applicant: Atopia Therapeutics SA. Application EP. The sequence listing filed with the application follows.

SEQUENCE LISTING (43 sequences)

SEQ ID NO: 1 - protein, 765 aa, synthetic construct
  VARIANT 1: note = X1 is absent.
  VARIANT 5: note = X2 is selected from Threonine, Methionine, or a homologous variant thereof.
  VARIANT 20: note = X3 is selected from Threonine, Alanine, or a homologous variant thereof.
  VARIANT 21: note = X4 is selected from Alanine, Threonine, or a homologous variant thereof.
  VARIANT 30: note = X5 is selected from Glycine, Serine, Alanine, or a homologous variant thereof.
  VARIANT 31: note = X6 is selected from Tryptophan, Glycine, or a homologous variant thereof.
  VARIANT 32: note = X7 is selected from Glycine, Glutamate, or a homologous variant thereof.
  VARIANT 35: note = X8 is selected from Glutamine, Proline, Lysine, or a homologous variant thereof.
  VARIANT 36: note = X9 is selected from Alanine, Serine, or a homologous variant thereof.
  VARIANT 38: note = X10 is selected from Glutamate, Glutamine, or a homologous variant thereof.
  VARIANT 42: note = X11 is selected from Threonine, Asparagine, Isoleucine, Alanine, Proline, Serine, or a homologous variant thereof.
  VARIANT 43: note = X12 is selected from Proline, Glutamine, Threonine, or a homologous variant thereof.
  VARIANT 45: note = X13 is selected from Lysine, Threonine, or a homologous variant thereof.
  VARIANT 47: note = X14 is selected from Aspartate, Glutamate, Asparagine, Lysine, or a homologous variant thereof.
  VARIANT 50: note = X15 is selected from Tryptophan, Arginine, or a homologous variant thereof.
  VARIANT 51: note = X16 is selected from Arginine, Histidine, or a homologous variant thereof.
  VARIANT 54: note = X17 is selected from Alaine, Threonine, or a homologous variant thereof.
  VARIANT 55: note = X18 is selected from Glycine, Arginine, or a homologous variant thereof.
  VARIANT 56: note = X19 is selected from Lysine, Arginine, Isoleucine, Serine, Asparagine, or a homologous variant thereof.
  VARIANT 59: note = X20 is selected from Asparagine, Aspartate, or a homologous variant thereof.
  VARIANT 60: note = X21 is selected from Glutamate, Asparagine, Glutamine, Histidine, Serine, Aspartate, or a homologous variant thereof.
  VARIANT 62: note = X22 is selected from Proline, Leucine, Threonine, Serine, or a homologous variant thereof.
  VARIANT 63: note = X23 is selected from Asparagine, Histidine, Threonine, Serine, Lysine, or a homologous variant thereof.
  VARIANT 64: note = X24 is selected from Lysine, Glycine, or a homologous variant thereof.
  VARIANT 65: note = X25 is selected from Glutamate, Glutamine, or a homologous variant thereof.
  VARIANT 67: note = X26 is selected from Aspartate, Glycine, or a homologous variant thereof.
  VARIANT 70: note = X27 is selected from Lysine, Glutamine, Arginine, Threonine, or a homologous variant thereof.
  VARIANT 71: note = X28 is selected from Serine, Alanine, or a homologous variant thereof.
  VARIANT 75: note = X29 is selected from Serine, Asparagine, or a homologous variant thereof.
  VARIANT 78: note = X30 is selected from Aspartate, Asparagine, Histidine, Glutamate, or a homologous variant thereof.
  VARIANT 79: note = X31 is selected from Glycine, Tryptophan, or a homologous variant thereof.
  VARIANT 83: note = X32 is selected from Tryptophan, Tyrosine, Leucine, or a homologous variant thereof.
  VARIANT 86: note = X33 is selected from Alanine, Threonine, Valine, or a homologous variant thereof.
  VARIANT 87: note = X34 is selected from Alaine, Serine, Threonine, or a homologous variant thereof.
  VARIANT 88: note = X35 is selected from Arginine, Threonine, Glycine, Lysine, Asparagine, Serine, or a homologous variant thereof.
  VARIANT 94: note = X36 is selected from Glycine, Aspartate, Serine, or a homologous variant thereof.
  VARIANT 97: note = X37 is selected from Tryptophan, Glutamine, Arginine, Leucine, Serine, or a homologous variant thereof.
  VARIANT 102: note = X38 is selected from Valine, Methionine, or a homologous variant thereof.
  VARIANT 103: note = X39 is selected from Aspartate, Asparagine, Glycine, or a homologous variant thereof.
  VARIANT 105: note = X40 is selected from Lysine, Glutamine, Glutamate, or a homologous variant thereof.
  VARIANT 106: note = X41 is selected from Aspartate, Asparagine, or a homologous variant thereof.
  VARIANT 107: note = X42 is selected from Alanine, Serine, or a homologous variant thereof.
  VARIANT 110: note = X43 is selected from Threonine, Alanine, or a homologous variant thereof.
  VARIANT 112: note = X44 is selected from Lysine, Asparagine, Threonine, or a homologous variant thereof.
  VARIANT 117: note = X45 is selected from Arginine, Isoleucine, Lysine, or a homologous variant thereof.
  VARIANT 125: note = X46 is selected from Aspartate, Asparagine, or a homologous variant thereof.
  VARIANT 126: note = X47 is selected from Valine, Isoleucine, Methionine, or a homologous variant thereof.
  VARIANT 134: note = X48 is selected from Arginine, Histidine, or a homologous variant thereof.
  VARIANT 148: note = X49 is selected from Aspartate, Glycine, or a homologous variant thereof.
  VARIANT 149: note = X50 is selected from Serine, Alanine, Glycine, Asparagine, Lysine, or a homologous variant thereof.
  VARIANT 150: note = X51 is selected from Alanine, Threonine, or a homologous variant thereof.
  VARIANT 151: note = X52 is selected from Aspartate, Asparagine, or a homologous variant thereof.
  VARIANT 157: note = X53 is selected from Aspartate, Asparagine, or a homologous variant thereof.
  VARIANT 159: note = X54 is selected from Asparagine, Aspartate, Serine, or a homologous variant thereof.
  VARIANT 161: note = X55 is selected from Lysine, Histidine, or a homologous variant thereof.
  VARIANT 164: note = X56 is selected from Serine, Leucine, or a homologous variant thereof.
  VARIANT 165: note = X57 is selected from Isoleucine, Methionine, Valine, or a homologous variant thereof.
  VARIANT 166: note = X58 is selected from Aspartate, Glutamate, Asparagine, or a homologous variant thereof.
  VARIANT 179: note = X59 is selected from Alaine, Threonine, or a homologous variant thereof.
  VARIANT 181: note = X60 is selected from Arginine, Methionine, or a homologous variant thereof.
  VARIANT 187: note = X61 is selected from Serine, Arginine, Glycine, or a homologous variant thereof.
  VARIANT 191: note = X62 is selected from Glutamine, Leucine, Lysine, or a homologous variant thereof.
  VARIANT 192: note = X63 is selected from Alanine, Serine, or a homologous variant thereof.
  VARIANT 193: note = X64 is selected from Serine, Glutamine, or a homologous variant thereof.
  VARIANT 194: note = X65 is selected from Glutamate, Glutamine, Lysine, or a homologous variant thereof.
  VARIANT 195: note = X66 is selected from Glycine, Lysine and Arginine, or a homologous variant thereof.
  VARIANT 197: note = X67 is selected from Threonine, Lysine, or a homologous variant thereof.
  VARIANT 198: note = X68 is selected from Serine, Glycine, or a homologous variant thereof.
  VARIANT 199: note = X69 is selected from Serine, Glycine, Aspartate, Arginine, Asparagine, or a homologous variant thereof.
  VARIANT 200: note = X70 is selected from Lysine, Glutamate, or a homologous variant thereof.
  VARIANT 202: note = X71 is selected from Alanine, Threonine, or a homologous variant thereof.
  VARIANT 210: note = X72 is selected from Alanine, Threonine, or a homologous variant thereof.
  VARIANT 211: note = X73 is selected from Threonine, Methionine, or a homologous variant thereof.
  VARIANT 213: note = X74 is absent or present and when present is selected from Asparagine or Tyrosine, or a homologous variant thereof.
  VARIANT 215: note = X75 is selected from Alanine or Valine, or a homologous variant thereof.
  VARIANT 216: note = X76 is selected from Serine, Glutamine, or a homologous variant thereof.
  VARIANT 217: note = X77 is selected from Asparagine, Serine, Lysine, or a homologous variant thereof.
  VARIANT 218: note = X78 is absent or present and when present is a peptide sequence Insert X78 or a homologous variant thereof.
  VARIANT 221: note = X79 is selected from Lysine, Aspartate, Asparagine, or a homologous variant thereof.
  VARIANT 223: note = X80 is selected from Methionine, Asparagine, Tyrosine, Tryptophan, or a homologous variant thereof.
  VARIANT 225: note = X81 is selected from Asparagine, Lysine, Histidine, or a homologous variant thereof.
  VARIANT 227: note = X82 is selected from Tryptophan, Leucine, or a homologous variant thereof.
  VARIANT 230: note = X83 is selected from Arginine, Leucine, or a homologous variant thereof.
  VARIANT 238: note = X84 is selected from Leucine, Phenylalanine, or a homologous variant thereof.
  VARIANT 240: note = X85 is selected from Proline, Leucine, or a homologous variant thereof.
  VARIANT 241: note = X86 is selected from Serine, Histidine, or a homologous variant thereof.
  VARIANT 242: note = X87 is selected from Tyrosine, Threonine, or a homologous variant thereof.
  VARIANT 246: note = X88 is selected from Asparagine, Aspartate, or a homologous variant thereof.
  VARIANT 247: note = X89 is selected from Threonine, Alanine, or a homologous variant thereof.
  VARIANT 248: note = X90 is selected from Serine, Leucine, or a homologous variant thereof.
  VARIANT 251: note = X91 is selected from Threonine, Alanine, Valine, Isoleucine, Glutamine, Glutamate, Lysine, or a homologous variant thereof.
  VARIANT 253: note = X92 is selected from Glutamate, Glutamine, or a homologous variant thereof.
  VARIANT 254: note = X93 is selected from Valine, Alanine, Methionine, Threonine, or a homologous variant thereof.
  VARIANT 255: note = X94 is selected from Asparagine, Aspartate, Histidine, Serine, or a homologous variant thereof.
  VARIANT 257: note = X95 is selected from Asparagine, Arginine, Serine, Aspartate, Threonine, or a homologous variant thereof.
  VARIANT 260: note = X96 is selected from Threonine, Alanine, Valine, Leucine, or a homologous variant thereof.
  VARIANT 261: note = X97 is selected from Valine, Alanine, Leucine, or a homologous variant thereof.
  VARIANT 263: note = X98 is selected from Aspartate, Asparagine, or a homologous variant thereof.
  VARIANT 264: note = X99 is selected from Lysine, Arginine, Glutamine, Histidine, Serine, or a homologous variant thereof.
  VARIANT 266: note = X100 is selected from Alanine, Threonine, Asparagine, Serine, Glycine, or a homologous variant thereof.
  VARIANT 268: note = X101 is selected from Glutamine, Tyrosine, or a homologous variant thereof.
  VARIANT 269: note = X102 is selected from Alanine, Valine, Glycine, or a homologous variant thereof.
  VARIANT 273: note = X103 is selected from Alanine, Leucine, Proline, or a homologous variant thereof.
  VARIANT 274: note = X104 is selected from Serine, Proline, Asparagine, Glycine, or a homologous variant thereof.
  VARIANT 275: note = X105 is selected from Asparagine, Lysine, Valine, or a homologous variant thereof.
  VARIANT 276: note = X106 is selected from Lysine, Arginine, Threonine, or a homologous variant thereof.
  VARIANT 277: note = X107 is selected from Threonine, Leucine, or a homologous variant thereof.
  VARIANT 278: note = X108 is selected from Histidine, Tyrosine, Asparagine, or a homologous variant thereof.
  VARIANT 280: note = X109 is selected from Glycine, Serine, or a homologous variant thereof.
  VARIANT 281: note = X110 is selected from Threonine, Valine, Alanine, or a homologous variant thereof.
  VARIANT 293: note = X111 is selected from Aspartate, Asparagine, or a homologous variant thereof.
  VARIANT 287: note = X112 is selected from Serine, Asparagine, or a homologous variant thereof.
  VARIANT 288: note = X113 is selected from Alanine, Valine, Threonine, or a homologous variant thereof.
  VARIANT 291: note = X114 is selected from asparagine, Serine, or a homologous variant thereof.
  VARIANT 294: note = X115 is selected from Alanine, Threonine, or a homologous variant thereof.
  VARIANT 296: note = X116 is selected from Proline, Glutamine, or a homologous variant thereof.
  VARIANT 297: note = X117 is absent.
  VARIANT 299: note = X118 is selected from Glycine, Alanine, or a homologous variant thereof.
  VARIANT 300: note = X119 is selected from Lysine, Glutamine, or a homologous variant thereof.
  VARIANT 301: note = X120 is selected from Aspartate, Asparagine, or a homologous variant thereof.
  VARIANT 303: note = X121 is selected from Valine, Alanine, Methionine, Isoleucine, or a homologous variant thereof.
  VARIANT 305: note = X122 is selected from Asparagine, Threonine, Asparagine, or a homologous variant thereof.
  VARIANT 307: note = X123 is selected from Asparagine, Aspartate, Phenylalanine, Serine, or a homologous variant thereof.
  VARIANT 308: note = X124 is selected from Arginine, Histidine, Serine, or a homologous variant thereof.
  VARIANT 310: note = X125 is selected from Asparagine, Serine, or a homologous variant thereof.
  VARIANT 312: note = X126 is selected from Asparagine, Lysine, Serine, or a homologous variant thereof.
  VARIANT 313: note = X127 is selected from Alaine, Serine, Threonine, or a homologous variant thereof.
  VARIANT 323: note = X128 is selected from Lysine, Threonine, or a homologous variant thereof.
  VARIANT 325: note = X129 is selected from Serine, Leucine, or a homologous variant thereof.
  VARIANT 332: note = X130 is selected from Histidine, Asparagine, Serine, Aspartate, or a homologous variant thereof.
  VARIANT 333: note = X131 is selected from Leucine, Phenylalanine, or a homologous variant thereof.
  VARIANT 334: note = X132 is selected from Asparagine, Histidine, Tyrosine, Alanine, Aspartate, or a homologous variant thereof.
  VARIANT 337: note = X133 is selected from Lysine, Glutamate, Glutamine, or a homologous variant thereof.
  VARIANT 338: note = X134 is selected from Glycine, Missing, or a homologous variant thereof.
  VARIANT 339: note = X135 is selected from Glycine, Alanine, or a homologous variant thereof.
  VARIANT 345: note = X136 is selected from Glutamine, Serine, or a homologous variant thereof.
  VARIANT 349: note = X138 is selected from Arginine, Histidine, or a homologous variant thereof.
  VARIANT 350: note = X139 is selected from Serine, Threonine, Leucine, or a homologous variant thereof.
  VARIANT 356: note = X140 is selected from Leucine, Isoleucine, Arginine, or a homologous variant thereof.
  VARIANT 359: note = X141 is selected from Asparagine, Aspartate, or a homologous variant thereof.
  VARIANT 363: note = X142 is selected from Aspartate, Asparagine, Glutamate, Serine, or a homologous variant thereof.
  VARIANT 365: note = X143 is selected from Proline, Alanine, Threonine, Serine, Leucine, or a homologous variant thereof.
  VARIANT 367: note = X144 is selected from Arginine, Methionine, Lysine, Glutamate, or a homologous variant thereof.
  VARIANT 370: note = X145 is selected from Asparagine, Glycine, Aspartate, or a homologous variant thereof.
  VARIANT 372: note = X146 is selected from Valine, Alanine, Glycine, or a homologous variant thereof.
  VARIANT 373: note = X147 is selected from Glycine, Serine, or a homologous variant thereof.
  VARIANT 375: note = X148 is selected from Tyrosine, Alanine, Serine, or a homologous variant thereof.
  VARIANT 376: note = X149 is selected from Alanine, Threonine, or a homologous variant thereof.
  VARIANT 378: note = X150 is selected from Alanine, Serine, Glutamine, or a homologous variant thereof.
  VARIANT 381: note = X151 is selected from Serine, Asparagine, or a homologous variant thereof.
  VARIANT 382: note = X152 is selected from Alanine, Threonine, or a homologous variant thereof.
  VARIANT 383: note = X153 is selected from Asparagine, Serine, or a homologous variant thereof.
  VARIANT 390: note = X154 is selected from Valine, Threonine, Alanine, Glutamate, or a homologous variant thereof.
  VARIANT 391: note = X155 is selected from Aspartate, Asparagine, or a homologous variant thereof.
  VARIANT 393: note = X156 is selected from Lysine, Asparagine, or a homologous variant thereof.
  VARIANT 394: note = X157 is selected from Asparagine, Lysine, Glutamine, or a homologous variant thereof.
  VARIANT 395: note = X158 is selected from Glycine, Alanine, Serine, or a homologous variant thereof.
  VARIANT 396: note = X159 is selected from Threonine, Isoleucine, or a homologous variant thereof.
  VARIANT 397: note = X160 is selected from Alanine, Isoleucine, Valine, or a homologous variant thereof.
  VARIANT 398: note = X161 is selected from Threonine, Alanine, or a homologous variant thereof.
  VARIANT 401: note = X162 is selected from Asparagine, Serine, Threonine, or a homologous variant thereof.
  VARIANT 402: note = X163 is selected from Aspartate, Asparagine, Isoleucine, Glutamate, or a homologous variant thereof.
  VARIANT 404: note = X164 is selected from Serine, Histidine, Asparagine, or a homologous variant thereof.
  VARIANT 406: note = X165 is selected from Glycine, Arginine, or a homologous variant thereof.
  VARIANT 408: note = X166 is selected from Phenylalanine, Alanine, Leucine, Serine, or a homologous variant thereof.
  VARIANT 409: note = X167 is selected from Valine, Glycine, or a homologous variant thereof.
  VARIANT 412: note = X168 is selected from Lysine, Arginine, Serine, Glutamate, or a homologous variant thereof.
  VARIANT 413: note = X169 is selected from Valine, Alanine, Leucine, Threonine, or a homologous variant thereof.
  VARIANT 414: note = X170 is selected from Aspartate, Serine, Asparagine, or a homologous variant thereof.
  VARIANT 415: note = X171 is selected from Alanine, Serine, or a homologous variant thereof.
  VARIANT 416: note = X172 is selected from Histidine, Tyrosine, Arginine, or a homologous variant thereof.
  VARIANT 418: note = X173 is absent or present and when present is a peptide sequence of SEQ ID NO: 6 or a homologous variant thereof.
  VARIANT 419: note = X174 is selected from Alanine, Threonine, Valine, or a homologous variant thereof.
  VARIANT 420: note = X175 is selected from Asparagine, Lysine, Tyrosine, Histidine, Isoleucine, or a homologous variant thereof.
  VARIANT 421: note = X176 is selected from Phenylalanine, Leucine, or a homologous variant thereof.
  VARIANT 422: note = X177 is selected from Lysine, Asparagine, Glutamine, Threonine, Glycine, or a homologous variant thereof.
  VARIANT 423: note = X178 is selected from Glycine, Aspartate, Glutamate, Lysine, Asparagine, or a homologous variant thereof.
  VARIANT 424: note = X179 is selected from Isoleucine, Lysine, Leucine, Tryptophan, or a homologous variant thereof.
  VARIANT 425: note = X180 is selected from Aspartate, Asparagine, Isoleucine, or a homologous variant thereof.
  VARIANT 426: note = X181 is selected from Alanine, Serine, Threonine, Methionine, or a homologous variant thereof.
  VARIANT 427: note = X182 is absent or present and when present is a peptide sequence Insert X182 or a homologous variant thereof.
  VARIANT 428: note = X183 is selected from Glycine, Serine, or a homologous variant thereof.
  VARIANT 429: note = X184 is selected from Aspartate, Asparagine, Serine, Methionine, or a homologous variant thereof.
  VARIANT 430: note = X185 is selected from Glycine, Asparagine, or a homologous variant thereof.
  VARIANT 433: note = X186 is selected from Asparagine, Threonine, Glycine, or a homologous variant thereof.
  VARIANT 434: note = X187 is absent or present and when present is a peptide sequence Insert X187 or a homologous variant thereof.
  VARIANT 435: note = X188 is selected from Threonine, Alanine, Serine, Leucine, Asparagine, or a homologous variant thereof.
  VARIANT 437: note = X189 is selected from Aspartate, Asparagine, Histidine, Serine, or a homologous variant thereof.
  VARIANT 439: note = X190 is selected from Serine, Cysteine, Asparagine, or a homologous variant thereof.
  VARIANT 440: note = X191 is selected from Glycine, Serine, or a homologous variant thereof.
  VARIANT 443: note = X192 is selected from Asparagine, Aspartate, Glycine, or a homologous variant thereof.
  VARIANT 446: note = X193 is selected from Asparagine, Isoleucine, Serine, or a homologous variant thereof.
  VARIANT 448: note = X194 is selected from Asparagine, Serine, or a homologous variant thereof.
  VARIANT 449: note = X195 is selected from Lysine, Asparagine, or a homologous variant thereof.
  VARIANT 451: note = X196 is selected from Isoleucine, Threonine, Valine, or a homologous variant thereof.
  VARIANT 453: note = X197 is selected from Alanine, Serine, or a homologous variant thereof.
  VARIANT 454: note = X198 is selected from Serine, Alanine, or a homologous variant thereof.
  VARIANT 458: note = X199 is selected from Alanine, Asparagine, Valine, Serine, or a homologous variant thereof.
  VARIANT 461: note = X200 is selected from Asparagine, Threonine, or a homologous variant thereof.
  VARIANT 462: note = X201 is selected from Phenylalanine, Serine, or a homologous variant thereof.
  VARIANT 463: note = X202 is selected from Asparagine, Aspartate, Serine, Threonine, or a homologous variant thereof.
  VARIANT 465: note = X203 is selected from Asparagine, Lysine, or a homologous variant thereof.
  VARIANT 466: note = X204 is selected from Glutamate, Lysine, Aspartate, or a homologous variant thereof.
  VARIANT 470: note = X205 is selected from Lysine, Arginine, Threonine, or a homologous variant thereof.
  VARIANT 472: note = X206 is selected from Asparagine, Arginine, or a homologous variant thereof.
  VARIANT 473: note = X207 is selected from Glycine, Valine, or a homologous variant thereof.
  VARIANT 474: note = X208 is selected from Valine, Isoleucine, Leucine, Glutamine, or a homologous variant thereof.
  VARIANT 475: note = X209 is selected from Serine, Asparagine, or a homologous variant thereof.
  VARIANT 478: note = X210 is selected from Glutamate, Glutamine, or a homologous variant thereof.
  VARIANT 483: note = X212 is selected from Serine, Glycine, Aspartate, Alanine, or a homologous variant thereof.
  VARIANT 484: note = X213 is selected from Glutamate, Lysine, Glycine, Aspartate, or a homologous variant thereof.
  VARIANT 485: note = X214 is selected from Aspartate, Asparagine, Isoleucine, or a homologous variant thereof.
  VARIANT 488: note = X215 is selected from Serine, Asparagine, Aspartate, or a homologous variant thereof.
  VARIANT 489: note = X216 is selected from Glutamine, Glutamate, Lysine, or a homologous variant thereof.
  VARIANT 491: note = X217 is selected from Arginine, Histidine, Tyrosine, or a homologous variant thereof.
  VARIANT 493: note = X218 is selected from Asparagine, Glycine, Serine
  VARIANT 494: note = X219 is selected from Threonine, Alanine, Valine, Isoleucine, or a homologous variant thereof.
  VARIANT 496: note = X220 is selected from Arginine, Serine, or a homologous variant thereof.
  VARIANT 498: note = X221 is selected from Glutamate, Glutamine, or a homologous variant thereof.
  VARIANT 499: note = X222 is selected from Threonine, Methionine, or a homologous variant thereof.
  VARIANT 501: note = X223 is selected from Threonine, Tyrosine, Isoleucine, or a homologous variant thereof.
  VARIANT 502: note = X224 is selected from Arginine, Serine, or a homologous variant thereof.
  VARIANT 503: note = X225 is selected from Serine, Glutamine, Proline, or a homologous variant thereof.
  VARIANT 506: note = X226 is selected from Serine, Alanine, or a homologous variant thereof.
  VARIANT 510: note = X227 is selected from Lysine, Glutamine, Threonine, Arginine
  VARIANT 513: note = X228 is selected from Glycine, Serine, or a homologous variant thereof.
  VARIANT 515: note = X229 is selected from Glutamate, Lysine, Glutamine, or a homologous variant thereof.
  VARIANT 516: note = X230 is selected from Lysine, Asparagine, or a homologous variant thereof.
  VARIANT 518: note = X231 is selected from Valine, Aspartate
  VARIANT 520: note = X232 is selected from Aspartate, Asparagine, or a homologous variant thereof.
  VARIANT 523: note = X233 is selected from Tyrosine, Cysteine, Phenylalanine
  VARIANT 524: note = X234 is selected from Tyrosine, Histidine, or a homologous variant thereof.
  VARIANT 525: note = X235 is selected from Serine, Alanine, or a homologous variant thereof.
  VARIANT 533: note = X236 is selected from Arginine, Lysine, Serine, or a homologous variant thereof.
  VARIANT 534: note = X237 is selected from Asparagine, Serine, or a homologous variant thereof.
  VARIANT 536: note = X238 is selected from Lysine, Threonine, Arginine, or a homologous variant thereof.
  VARIANT 537: note = X239 is selected from Asparagine, Aspartate, Isoleucine, or a homologous variant thereof.
  VARIANT 541: note = X240 is selected from Threonine, Asparagine, Alanine, Isoleucine, or a homologous variant thereof.
  VARIANT 542: note = X241 is selected from Arginine, Asparagine, Lysine, Aspartate, Glycine, or a homologous variant thereof.
  VARIANT 545: note = X242 is selected from Alanine, Leucine, Threonine, or a homologous variant thereof.
  VARIANT 546: note = X243 is selected from Phenylalanine, Serine, or a homologous variant thereof.
  VARIANT 547: note = X244 is selected from Glycine, Serine, or a homologous variant thereof.
  VARIANT 548: note = X245 is selected from Threonine, Proline, Alanine, Serine, or a homologous variant thereof.
  VARIANT 549: note = X246 is selected from Proline, Glutamine, or a homologous variant thereof.
  VARIANT 550: note = X247 is selected from Glutamate, Glycine, or a homologous variant thereof.
  VARIANT 551: note = X248 is selected from Asparagine, Serine, Tyrosine, or a homologous variant thereof.
  VARIANT 552: note = X249 is selected from Isoleucine, Proline, or a homologous variant thereof.
  VARIANT 553: note = X250 is selected from Alanine, Tryptophan, Proline, Tyrosine, or a homologous variant thereof.
  VARIANT 555: note = X251 is selected from Lysine, Threonine, Isoleucine, Alanine, or a homologous variant thereof.
  VARIANT 556: note = X252 is selected from Threonine, Serine, Alanine, or a homologous variant thereof.
  VARIANT 557: note = X253 is selected from Glycine, Lysine, Glutamine, Asparagine, or a homologous variant thereof.
  VARIANT 559: note = X254 is selected from Methionine, Tyrosine, Threonine, or a homologous variant thereof.
  VARIANT 560: note = X255 is selected from Phenylalanine, Valine, Tyrosine, or a homologous variant thereof.
  VARIANT 564: note = X256 is selected from Threonine, Alanine, Serine, or a homologous variant thereof.
  VARIANT 566: note = X257 is selected from Asparagine, Glycine, Threonine, Alanine, Aspartate, or a homologous variant thereof.
  VARIANT 567: note = X258 is selected from Serine, Glutamine, Proline, Tyrosine, Histidine, Asparagine, Leucine, or a homologous variant thereof.
  VARIANT 570: note = X259 is selected from Serine, Valine, Isoleucine, Asparagine, Alanine, or a homologous variant thereof.
  VARIANT 572: note = X260 is selected from Aspartate, Asparagine, or a homologous variant thereof.
  VARIANT 574: note = X261 is selected from Glycine, Serine, Lysine, Asparagine, or a homologous variant thereof.
  VARIANT 575: note = X262 is selected from Lysine, Glutamine, Serine, or a homologous variant thereof.
  VARIANT 576: note = X263 is selected from Aspartate, Phenylalanine, Isoleucine, or a homologous variant thereof.
  VARIANT 577: note = X264 is selected from Leucine, Serine, Glutamine, or a homologous variant thereof.
  VARIANT 578: note = X265 is selected from Aspartate, Asparagine, or a homologous variant thereof.
  VARIANT 580: note = X266 is selected from Threonine, Alanine, or a homologous variant thereof.
  VARIANT 582: note = X267 is selected from Glutamine, Serine, Histidine, Tyrosine, or a homologous variant thereof.
  VARIANT 583: note = X268 is selected from Glycine, Glutamate, Arginine, or a homologous variant thereof.
  VARIANT 584: note = X269 is selected from Histidine, Asparagine, Aspartate, or a homologous variant thereof.
  VARIANT 586: note = X270 is selected from Threonine, Isoleucine, Valine, or a homologous variant thereof.
  VARIANT 589: note = X271 is selected from Glutamine, Arginine, or a homologous variant thereof.
  VARIANT 590: note = X272 is selected from Glycine, Alanine, Serine, or a homologous variant thereof.
  VARIANT 591: note = X273 is selected from Threonine, Leucine, Valine, Alanine, Isoleucine, or a homologous variant thereof.
  VARIANT 592: note = X274 is selected from Methionine, Isoleucine, Glutamine, or a homologous variant thereof.
  VARIANT 594: note = X275 is selected from Leucine, Tyrosine, or a homologous variant thereof.
  VARIANT 597: note = X276 is selected from Glutamine, Arginine, or a homologous variant thereof.
  VARIANT 598: note = X277 is selected from Aspartate, Glycine, Asparagine, or a homologous variant thereof.
  VARIANT 599: note = X278 is selected from Glycine, Arginine, or a homologous variant thereof.
  VARIANT 600: note = X279 is selected from Arginine, Lysine, Glutamine, Asparagine, or a homologous variant thereof.
  VARIANT 601: note = X280 is selected from Valine, Isoleucine, Threonine, or a homologous variant thereof.
  VARIANT 602: note = X281 is selected from Alanine, Glutamate, Glutamine, Lysine, or a homologous variant thereof.
  VARIANT 603: note = X282 is selected from Threonine, Alanine, or a homologous variant thereof.
  VARIANT 605: note = X283 is selected from Asparagine, Serine, Glycine, or a homologous variant thereof.
  VARIANT 607: note = X284 is selected from Glycine, Aspartate, or a homologous variant thereof.
  VARIANT 608: note = X285 is selected from Histidine, Lysine, Asparagine, Tyrosine, Aspartate, or a homologous variant thereof.
  VARIANT 609: note = X286 is selected from Glutamine, Alanine, Threonine, Valine, or a homologous variant thereof.
  VARIANT 610: note = X287 is selected from Alanine, Valine, Threonine, or a homologous variant thereof.
  VARIANT 611: note = X288 is selected from Serine, Threonine, Alanine, Valine, or a homologous variant thereof.
  VARIANT 613: note = X289 is selected from Isoleucine, Methionine, Lysine, Valine, Serine, Leucine, Phenylalanine, Arginine, or a homologous variant thereof.
  VARIANT 615: note = X290 is selected from Asparagine, Serine, or a homologous variant thereof.
  VARIANT 617: note = X291 is selected from Leucine, Aspartate, Valine, Asparagine, Methionine, Glutamate, Serine, or a homologous variant thereof.
  VARIANT 620: note = X292 is selected from Serine, Asparagine, or a homologous variant thereof.
  VARIANT 621: note = X293 is selected from Alanine, Threonine, Serine, Methionine, or a homologous variant thereof.
  VARIANT 626: note = X294 is selected from Lysine, Glutamine, or a homologous variant thereof.
  VARIANT 628: note = X295 is selected from Leucine, Isoleucine, Serine, or a homologous variant thereof.
  VARIANT 630: note = X296 is selected from Lysine, Asparagine, Arginine, or a homologous variant thereof.
  VARIANT 632: note = X297 is selected from Asparagine, Aspartate, Threonine, or a homologous variant thereof.
  VARIANT 633: note = X298 is selected from Asparagine, Aspartate, Serine, or a homologous variant thereof.
  VARIANT 636: note = X299 is selected from Asparagine, Aspartate, or a homologous variant thereof.
  VARIANT 638: note = X300 is selected from Threonine, Isoleucine, Valine, or a homologous variant thereof.
  VARIANT 639: note = X301 is selected from Lysine, Glutamate, or a homologous variant thereof.
  VARIANT 641: note = X302 is selected from Lysine, Threonine, Arginine, Alanine, or a homologous variant thereof.
  VARIANT 642: note = X303 is selected from Glutamate, Lysine, or a homologous variant thereof.
  VARIANT 647: note = X304 is selected from Lysine, Arginine, Serine, or a homologous variant thereof.
  VARIANT 649: note = X305 is selected from Arginine, Glutamine, Lysine, Proline, or a homologous variant thereof.
  VARIANT 650: note = X306 is selected from Asparagine, Isoleucine, Valine, Threonine, or a homologous variant thereof.
  VARIANT 652: note = X307 is selected from Aspartate, Glycine, Asparagine, Serine, Arginine, or a homologous variant thereof.
  VARIANT 654: note = X308 is selected from Asparagine, Glycine, Glutamate, Aspartate, Valine, or a homologous variant thereof.
  VARIANT 655: note = X309 is selected from Leucine, Asparagine, or a homologous variant thereof.
  VARIANT 657: note = X310 is absent or present and when present is a peptide sequence Insert X310 or a homologous variant thereof.
  VARIANT 659: note = X311 is selected from Tyrosine, Threonine, Leucine, Glutamate, Alanine, Isoleucine, Valine, or a homologous variant thereof.
  VARIANT 660: note = X312 is selected from Aspartate, Glycine, or a homologous variant thereof.
  VARIANT 661: note = X313 is selected from Asparagine, Threonine, Serine, Alanine, Isoleucine, or a homologous variant thereof.
  VARIANT 662: note = X314 is selected from Isoleucine, Asparagine, Lysine, Valine, Threonine, Serine, Aspartate, Alanine, or a homologous variant thereof.
  VARIANT 663: note = X315 is selected from Serine, Glycine, Asparagine, Histidine, Arginine, Alanine, or a homologous variant thereof.
  VARIANT 664: note = X316 is selected from Alanine, Isoleucine, Threonine, Phenylalanine, Serine, Valine, Glutamine, Lysine, or a homologous variant thereof.
  VARIANT 665: note = X317 is selected from Serine, Asparagine, Histidine, Arginine, Alanine, Glycine, or a homologous variant thereof.
  VARIANT 666: note = X318 is selected from Asparagine, Glycine, Alanine, Methionine, Aspartate, Glutamate, or a homologous variant thereof.
  VARIANT 667: note = X319 is selected from Threonine, Valine, Alanine, Leucine, Isoleucine, or a homologous variant thereof.
  VARIANT 668: note = X320 is selected from Asparagine, Serine, Lysine, Isoleucine, Leucine, or a homologous variant thereof.
  VARIANT 669: note = X321 is selected from Leucine, Isoleucine, Proline, Glutamine, or a homologous variant thereof.
  VARIANT 670: note = X322 is selected from Glutamine, Glutamate, Methionine, Isoleucine, Leucine, or a homologous variant thereof.
  VARIANT 672: note = X323 is selected from Glutamine, Serine, Glutamate, or a homologous variant thereof.
  VARIANT 673: note = X324 is selected from Phenylalanine, Valine, or a homologous variant thereof.
  VARIANT 674: note = X325 is selected from Lysine, Asparagine, or a homologous variant thereof.
  VARIANT 675: note = X326 is selected from Glutamate, Glycine, Aspartate, or a homologous variant thereof.
  VARIANT 681: note = X327 is selected from Asparagine, Glutamate, or a homologous variant thereof.
  VARIANT 682: note = X328 is selected from Asparagine, Histidine, or a homologous variant thereof.
  VARIANT 688: note = X329 is selected from Threonine, Isoleucine, or a homologous variant thereof.
  VARIANT 692: note = X330 is selected from Arginine, Glutamine, or a homologous variant thereof.
  VARIANT 693: note = X331 is absent or present and when present is a peptide sequence Insert X331 or a homologous variant thereof.
  VARIANT 694: note = X332 is selected from Asparagine, Lysine, Aspartate, or a homologous variant thereof.
  VARIANT 695: note = X333 is selected from Threonine, Glutamate, Leucine, Isoleucine, or a homologous variant thereof.
  VARIANT 696: note = X334 is selected from Aspartate, Asparagine, or a homologous variant thereof.
  VARIANT 700: note = X335 is selected from Alanine, Valine, Threonine, Glutamine, or a homologous variant thereof.
  VARIANT 702: note = X336 is selected from Glycine, Tryptophan, or a homologous variant thereof.
  VARIANT 703: note = X337 is selected from Methionine, Threonine, Isoleucine, Lysine, Arginine, or a homologous variant thereof.
  VARIANT 707: note = X338 is selected from Asparagine, Aspartate, or a homologous variant thereof.
  VARIANT 708: note = X339 is selected from Glutamine, Threonine, Asparagine, or a homologous variant thereof.
  VARIANT 709: note = X340 is selected from Serine, Alanine, Aspartate, Glycine, Asparagine, or a homologous variant thereof.
  VARIANT 712: note = X341 is selected from Asparagine, Methionine, Serine, Threonine, or a homologous variant thereof.
  VARIANT 713: note = X342 is selected from Asparagine, Threonine, or a homologous variant thereof.
  VARIANT 715: note = X343 is selected from Aspartate, Glutamate, Asparagine, Serine, Lysine, Glycine, or a homologous variant thereof.
  VARIANT 716: note = X344 is selected from Asparagine, Lysine, Aspartate, Serine, or a homologous variant thereof.
  VARIANT 718: note = X345 is selected from Lysine, Arginine, Asparagine, Glutamate, or a homologous variant thereof.
  VARIANT 721: note = X346 is selected from Isoleucine, Glutamate, Leucine, Valine, Glycine, Lysine, or a homologous variant thereof.
  VARIANT 726: note = X347 is selected from Lysine, Arginine, Isoleucine, or a homologous variant thereof.
  VARIANT 728: note = X348 is selected from Isoleucine, Leucine, Threonine, or a homologous variant thereof.
  VARIANT 729: note = X349 is selected from Glycine, Serine, or a homologous variant thereof.
  VARIANT 731: note = X350 is selected from Serine, Asparagine, Aspartate, or a homologous variant thereof.
  VARIANT 733: note = X351 is selected from Threonine, Asparagine, Isoleucine, or a homologous variant thereof.
  VARIANT 735: note = X352 is selected from Asparagine, Aspartate, or a homologous variant thereof.
  VARIANT 736: note = X353 is selected from Glycine, Asparagine, Serine, Aspartate, Lysine, or a homologous variant thereof.
  VARIANT 739: note = X354 is selected from Lysine, Threonine, or a homologous variant thereof.
  VARIANT 740: note = X355 is selected from Serine, Alanine, Threonine, or a homologous variant thereof.
  VARIANT 742: note = X356 is selected from Tyrosine, Arginine, Histidine, Asparagine, Leucine, Serine, or a homologous variant thereof.
  VARIANT 743: note = X357 is selected from Tyrosine, Leucine, Valine, Phenylalanine, or a homologous variant thereof.
  VARIANT 744: note = X358 is selected from Leucine, Glycine, Arginine, or a homologous variant thereof.
  VARIANT 745: note = X359 is selected from Glycine, Asparagine, Lysine, Glutamine, or a homologous variant thereof.
  VARIANT 746: note = X360 is selected from Asparagine, Alanine, Aspartate, or a homologous variant thereof.
  VARIANT 747: note = X361 is selected from Serine, Alanine, Valine, Phenylalanine, Threonine, or a homologous variant thereof.
  VARIANT 748: note = X362 is selected from Threonine, Alanine, Tyrosine, or a homologous variant thereof.
  VARIANT 749: note = X363 is selected from Proline, Threonine, Leucine, Alanine, or a homologous variant thereof.
  VARIANT 750: note = X364 is selected from Threonine, Alanine, Serine, Proline, Asparagine, or a homologous variant thereof.
  VARIANT 751: note = X365 is selected from Glutamate, Aspartate, Threonine, Serine, Asparagine, or a homologous variant thereof.
  VARIANT 752: note = X366 is selected from Asparagine, Lysine, Serine, Aspartate, Proline, Glutamate, or a homologous variant thereof.
  VARIANT 753: note = X367 is selected from Glycine, Glutamate, Serine, Proline, Threonine, Asparagine, Aspartate, or a homologous variant thereof.
  VARIANT 754: note = X368 is selected from Glycine, Aspartate, Threonine, Serine, Valine, or a homologous variant thereof.
  VARIANT 755: note = X369 is selected from Asparagine, Aspartate, Serine, or a homologous variant thereof.
  VARIANT 756: note = X370 is selected from Threonine, Leucine, Isoleucine, Proline, or a homologous variant thereof.
  VARIANT 758: note = X371 is selected from Threonine, Proline, or a homologous variant thereof.
  VARIANT 759: note = X372 is selected from Asparagine, Aspartate, Lysine, Threonine, Serine, or a homologous variant thereof.
  VARIANT 760: note = X374 is selected from Proline, Alanine, Threonine, or a homologous variant thereof.
  VARIANT 761: note = X375 is selected from Threonine, Lysine, Glutamate, Asparagine, Tyrosine, or a homologous variant thereof.
  VARIANT 762: note = X376 is selected from Asparagine, Serine, or a homologous variant thereof.
  VARIANT 763: note = X377 is selected from Threonine, Alanine, Serine, Lysine, Proline, or a homologous variant thereof.
  VARIANT 764: note = X378 is selected from Threonine, Glutamate, Alanine, Proline, Serine, Isoleucine, Lysine, or a homologous variant thereof.
  VARIANT 765: note = X379 is absent or present and when present is a peptide sequence Insert X379 or a homologous variant thereof.
  VARIANT 481: note = X211 is selected from Histidine, Asparagine, Tyrosine, Isoleucine, or a homologous variant thereof.
  VARIANT 759: note = X373 is selected from Leucine, Asparagine, Phenylalanine, or a homologous variant thereof.
XAFFXTVIIPAIVGGIATGXXVGTVSGLLXXXLKXXEXANKXXDXPXKVXXIQXXXGFXXFXXXXYXLYXXLLSXKIXXGWDXGNXXXHYWVKXGQXNKLEXXMXXXVGXYXLSGLXNFTGGDLXXNMQKATLXLGQFNGNSFTSYKXXXXRTTRVXFXAXNIXXXNFVEINNRVGSGXGXKAXSTVLTLXXXXXIXXXXNXEISLYDGXXLXLXXXXSVXLXGXVXMGXLQYVGAYXAXXXSTIXXXKVXGXXXFXHLXXGXXNXAXXGIIXXXXXXIXXLXLWQXXGLXIIXPXXGXXXTXVXIXXIXTXXDGTIRVGGYXAXLTTNAAXXXIGXXXVNLSNXXSGXXLLVENXTGXITVXGXLXVNXQXXGXXLXGSXXXFEFKAGXXTXXXXXXFNXXIXLXRXXNLXXXXXTXXXXXXXXXXXXXGFXXXLXFXXVTXKVXIXXLXTXXTNVXVKXXXIXXLIVXTXXXXVGXYTXFXXXIGXXSXIXXVXLXXGXXXIFXGGVXFKXGXXLXIXEFXXXPWNYFDAXXIXXVEIXXKFXXXXXXXXXGXXXLXXNNLXLXXNAXMXYXXXXXLXIXXXFXNNXXXXNXLVXXXXXXXLXVXXXXXMXFXNXIDXXTGFYXPXIXIXXAQXLXXNXXHVLLXAXXIXYXXVXSXXXXXXXXXXXXEXXXXRLALYXXNNRMDXCVVXXXXXDIKXCXXAIGXXXMVXXPXXYXYLXGKAWXNXXIXKXAXXSXIXVXXXXXXXXXXXXXXXXXXXXXXXX

SEQ ID NO: 2 - protein, 765 aa, synthetic construct
  VARIANT 1: note = X1 is a peptide sequence of SEQ ID No: 3 or a homologous variant thereof.
  VARIANT 5: note = X2 is selected from Threonine, Methionine, or a homologous variant thereof.
  VARIANT 20: note = X3 is selected from Threonine, Alanine, or a homologous variant thereof.
  VARIANT 21: note = X4 is selected from Alanine, Threonine, or a homologous variant thereof.
  VARIANT 35: note = X8 is selected from Glutamine, Proline, Lysine, or a homologous variant thereof.
  VARIANT 38: note = X10 is selected from Glutamate, Glutamine, or a homologous variant thereof.
  VARIANT 42: note = X11 is selected from Threonine, Asparagine, Isoleucine, Alanine, Proline, Serine, or a homologous variant thereof.
  VARIANT 45: note = X13 is selected from Lysine, Threonine, or a homologous variant thereof.
  VARIANT 47: note = X14 is selected from Aspartate, Glutamate, Asparagine, Lysine, or a homologous variant thereof.
  VARIANT 50: note = X15 is selected from Tryptophan, Arginine, or a homologous variant thereof.
  VARIANT 51: note = X16 is selected from Arginine, Histidine, or a homologous variant thereof.
  VARIANT 56: note = X19 is selected from Lysine, Arginine, Isoleucine, Serine, Asparagine, or a homologous variant thereof.
  VARIANT 59: note = X20 is selected from Asparagine, Aspartate, or a homologous variant thereof.
  VARIANT 60: note = X21 is selected from Glutamate, Asparagine, Glutamine, Histidine, Serine, Aspartate, or a homologous variant thereof.
  VARIANT 62: note = X22 is selected from Proline, Leucine, Threonine, Serine, or a homologous variant thereof.
  VARIANT 63: note = X23 is selected from Asparagine, Histidine, Threonine, Serine, Lysine, or a homologous variant thereof.
  VARIANT 65: note = X25 is selected from Glutamate, Glutamine, or a homologous variant thereof.
  VARIANT 70: note = X27 is selected from Lysine, Glutamine, Arginine, Threonine, or a homologous variant thereof.
  VARIANT 78: note = X30 is selected from Aspartate, Asparagine, Histidine, Glutamate, or a homologous variant thereof.
  VARIANT 83: note = X32 is selected from Tryptophan, Tyrosine, Leucine, or a homologous variant thereof.
  VARIANT 94: note = X36 is selected from Glycine, Aspartate, Serine, or a homologous variant thereof.
  VARIANT 103: note = X39 is selected from Aspartate, Asparagine, Glycine, or a homologous variant thereof.
  VARIANT 105: note = X40 is selected from Lysine, Glutamine, Glutamate, or a homologous variant thereof.
  VARIANT 106: note = X41 is selected from Aspartate, Asparagine, or a homologous variant thereof.
  VARIANT 112: note = X44 is selected from Lysine, Asparagine, Threonine, or a homologous variant thereof.
  VARIANT 117: note = X45 is selected from Arginine, Isoleucine, Lysine, or a homologous variant thereof.
  VARIANT 126: note = X47 is selected from Valine, Isoleucine, Methionine, or a homologous variant thereof.
  VARIANT 149: note = X50 is selected from Serine, Alanine, Glycine, Asparagine, Lysine, or a homologous variant thereof.
  VARIANT 150: note = X51 is selected from Alanine, Threonine, or a homologous variant thereof.
  VARIANT 151: note = X52 is selected from Aspartate, Asparagine, or a homologous variant thereof.
  VARIANT 157: note = X53 is selected from Aspartate, Asparagine, or a homologous variant thereof.
  VARIANT 159: note = X54 is selected from Asparagine, Aspartate, Serine, or a homologous variant thereof.
  VARIANT 164: note = X56 is selected from Serine, Leucine, or a homologous variant thereof.
  VARIANT 191: note = X62 is selected from Glutamine, Leucine, Lysine, or a homologous variant thereof.
  VARIANT 192: note = X63 is selected from Alanine, Serine, or a homologous variant thereof.
  VARIANT 194: note = X65 is selected from Glutamate, Glutamine, Lysine, or a homologous variant thereof.
  VARIANT 195: note = X66 is selected from Glycine, Lysine and Arginine, or a homologous variant thereof.
  VARIANT 197: note = X67 is selected from Threonine, Lysine, or a homologous variant thereof.
  VARIANT 200: note = X69 is selected from Serine, Glycine, Aspartate, Arginine, Asparagine, or a homologous variant thereof.
  VARIANT 199: note = X70 is selected from Lysine, Glutamate, or a homologous variant thereof.
  VARIANT 216: note = X76 is selected from Serine, Glutamine, or a homologous variant thereof.
  VARIANT 218: note = X78 is absent or present and when present is a peptide sequence Insert X78 or a homologous variant thereof.
  VARIANT 221: note = X79 is selected from Lysine, Aspartate, Asparagine, or a homologous variant thereof.
  VARIANT 223: note = X80 is selected from Methionine, Asparagine, Tyrosine, Tryptophan, or a homologous variant thereof.
  VARIANT 225: note = X81 is selected from Asparagine, Lysine, Histidine, or a homologous variant thereof.
  VARIANT 246: note = X88 is selected from Asparagine, Aspartate, or a homologous variant thereof.
  VARIANT 251: note = X91 is selected from Threonine, Alanine, Valine, Isoleucine, Glutamine, Glutamate, Lysine, or a homologous variant thereof.
  VARIANT 254: note = X93 is selected from Valine, Alanine, Methionine, Threonine, or a homologous variant thereof.
  VARIANT 257: note = X95 is selected from Asparagine, Arginine, Serine, Aspartate, Threonine, or a homologous variant thereof.
  VARIANT 260: note = X96 is selected from Threonine, Alanine, Valine, Leucine, or a homologous variant thereof.
  VARIANT 263: note = X98 is selected from Aspartate, Asparagine, or a homologous variant thereof.
  VARIANT 264: note = X99 is selected from Lysine, Arginine, Glutamine, Histidine, Serine, or a homologous variant thereof.
  VARIANT 266: note = X100 is selected from Alanine, Threonine, Asparagine, Serine, Glycine, or a homologous variant thereof.
  VARIANT 274: note = X104 is selected from Serine, Proline, Asparagine, Glycine, or a homologous variant thereof.
  VARIANT 275: note = X105 is selected from Asparagine, Lysine, Valine, or a homologous variant thereof.
  VARIANT 278: note = X108 is selected from Histidine, Tyrosine, Asparagine, or a homologous variant thereof.
  VARIANT 281: note = X110 is selected from Threonine, Valine, Alanine, or a homologous variant thereof.
  VARIANT 288: note = X113 is selected from Alanine, Valine, Threonine, or a homologous variant thereof.
  VARIANT 291: note = X114 is selected from asparagine, Serine, or a homologous variant thereof.
  VARIANT 294: note = X115 is selected from Alanine, Threonine, or a homologous variant thereof.
  VARIANT 297: note = X117 is absent.
  VARIANT 301: note = X120 is selected from Aspartate, Asparagine, or a homologous variant thereof.
  VARIANT 307: note = X123 is selected from Asparagine, Aspartate, Phenylalanine, Serine, or a homologous variant thereof.
  VARIANT 308: note = X124 is selected from Arginine, Histidine, Serine, or a homologous variant thereof.
  VARIANT 312: note = X126 is selected from Asparagine, Lysine, Serine, or a homologous variant thereof.
  VARIANT 313: note = X127 is selected from Alaine, Serine, Threonine, or a homologous variant thereof.
  VARIANT 332: note = X130 is selected from Histidine, Asparagine, Serine, Aspartate, or a homologous variant thereof.
  VARIANT 334: note = X132 is selected from Asparagine, Histidine, Tyrosine, Alanine, Aspartate, or a homologous variant thereof.
  VARIANT 337: note = X133 is selected from Lysine, Glutamate, Glutamine, or a homologous variant thereof.
  VARIANT 345: note = X136 is selected from Glutamine, Serine, or a homologous variant thereof.
  VARIANT 346: note = X137 is selected from Alanine, Threonine, Valine, or a homologous variant thereof.
  VARIANT 350: note = X139 is selected from Serine, Threonine, Leucine, or a homologous variant thereof.
  VARIANT 359: note = X141 is selected from Asparagine, Aspartate, or a homologous variant thereof.
  VARIANT 363: note = X142 is selected from Aspartate, Asparagine, Glutamate, Serine, or a homologous variant thereof.
  VARIANT 365: note = X143 is selected from Proline, Alanine, Threonine, Serine, Leucine, or a homologous variant thereof.
  VARIANT 372: note = X146 is selected from Valine, Alanine, Glycine, or a homologous variant thereof.
  VARIANT 375: note = X148 is selected from Tyrosine, Alanine, Serine, or a homologous variant thereof.
  VARIANT 376: note = X149 is selected from Alanine, Threonine, or a homologous variant thereof.
  VARIANT 382: note = X152 is selected from Alanine, Threonine, or a homologous variant thereof.
  VARIANT 390: note = X154 is selected from Valine, Threonine, Alanine, Glutamate, or a homologous variant thereof.
  VARIANT 391: note = X155 is selected from Aspartate, Asparagine, or a homologous variant thereof.
  VARIANT 395: note = X158 is selected from Glycine, Alanine, Serine, or a homologous variant thereof.
  VARIANT 402: note = X163 is selected from Aspartate, Asparagine, Isoleucine, Glutamate, or a homologous variant thereof.
  VARIANT 408: note = X166 is selected from Phenylalanine, Alanine, Leucine, Serine, or a homologous variant thereof.
  VARIANT 412: note = X168 is selected from Lysine, Arginine, Serine, Glutamate, or a homologous variant thereof.
  VARIANT 416: note = X172 is selected from Histidine, Tyrosine, Arginine, or a homologous variant thereof.
  VARIANT 418: note = X173 is absent or present and when present is a peptide sequence of SEQ ID NO: 6 or a homologous variant thereof.
  VARIANT 419: note = X174 is selected from Alanine, Threonine, Valine, or a homologous variant thereof.
  VARIANT 423: note = X178 is selected from Glycine, Aspartate, Glutamate, Lysine, Asparagine, or a homologous variant thereof.
  VARIANT 426: note = X181 is selected from Alanine, Serine, Threonine, Methionine, or a homologous variant thereof.
  VARIANT 427: note = X182 is absent or present and when present is a peptide sequence Insert X182 or a homologous variant thereof.
  VARIANT 434: note = X187 is absent or present and when present is a peptide sequence Insert X187 or a homologous variant thereof.
  VARIANT 435: note = X188 is selected from Threonine, Alanine, Serine, Leucine, Asparagine, or a homologous variant thereof.
  VARIANT 443: note = X192 is selected from Asparagine, Aspartate, Glycine, or a homologous variant thereof.
  VARIANT 446: note = X193 is selected from Asparagine, Isoleucine, Serine, or a homologous variant thereof.
  VARIANT 453: note = X197 is selected from Alanine, Serine, or a homologous variant thereof.
  VARIANT 458: note = X199 is selected from Alanine, Asparagine, Valine, Serine, or a homologous variant thereof.
  VARIANT 483: note = X212 is selected from Serine, Glycine, Aspartate, Alanine, or a homologous variant thereof.
  VARIANT 484: note = X213 is selected from Glutamate, Lysine, Glycine, Aspartate, or a homologous variant thereof.
  VARIANT 485: note = X214 is selected from Aspartate, Asparagine, Isoleucine, or a homologous variant thereof.
  VARIANT 489: note = X216 is selected from Glutamine, Glutamate, Lysine, or a homologous variant thereof.
  VARIANT 491: note = X217 is selected from Arginine, Histidine, Tyrosine, or a homologous variant thereof.
  VARIANT 493: note = X218 is selected from Asparagine, Glycine, Serine
  VARIANT 494: note = X219 is selected from Threonine, Alanine, Valine, Isoleucine, or a homologous variant thereof.
  VARIANT 499: note = X222 is selected from Threonine, Methionine, or a homologous variant thereof.
  VARIANT 506: note = X226 is selected from Serine, Alanine, or a homologous variant thereof.
  VARIANT 513: note = X228 is selected from Glycine, Serine, or a homologous variant thereof.
  VARIANT 534: note = X237 is selected from Asparagine, Serine, or a homologous variant thereof.
  VARIANT 541: note = X240 is selected from Threonine, Asparagine, Alanine, Isoleucine, or a homologous variant thereof.
  VARIANT 551: note = X248 is selected from Asparagine, Serine, Tyrosine, or a homologous variant thereof.
  VARIANT 553: note = X250 is selected from Alanine, Tryptophan, Proline, Tyrosine, or a homologous variant thereof.
  VARIANT 564: note = X256 is selected from Threonine, Alanine, Serine, or a homologous variant thereof.
  VARIANT 566: note = X257 is selected from Asparagine, Glycine, Threonine, Alanine, Aspartate, or a homologous variant thereof.
  VARIANT 567: note = X258 is selected from Serine, Glutamine, Proline, Tyrosine, Histidine, Asparagine, Leucine, or a homologous variant thereof.
  VARIANT 570: note = X259 is selected from Serine, Valine, Isoleucine, Asparagine, Alanine, or a homologous variant thereof.
  VARIANT 582: note = X267 is selected from Glutamine, Serine, Histidine, Tyrosine, or a homologous variant thereof.
  VARIANT 583: note = X268 is selected from Glycine, Glutamate, Arginine, or a homologous variant thereof.
  VARIANT 584: note = X269 is selected from Histidine, Asparagine, Aspartate, or a homologous variant thereof.
  VARIANT 589: note = X271 is selected from Glutamine, Arginine, or a homologous variant thereof.
  VARIANT 590: note = X272 is selected from Glycine, Alanine, Serine, or a homologous variant thereof.
  VARIANT 591: note = X273 is selected from Threonine, Leucine, Valine, Alanine, Isoleucine, or a homologous variant thereof.
  VARIANT 598: note = X277 is selected from Aspartate, Glycine, Asparagine, or a homologous variant thereof.
  VARIANT 599: note = X278 is selected from Glycine, Arginine, or a homologous variant thereof.
  VARIANT 603: note = X282 is selected from Threonine, Alanine, or a homologous variant thereof.
  VARIANT 607: note = X284 is selected from Glycine, Aspartate, or a homologous variant thereof.
  VARIANT 608: note = X285 is selected from Histidine, Lysine, Asparagine, Tyrosine, Aspartate, or a homologous variant thereof.
  VARIANT 609: note = X286 is selected from Glutamine, Alanine, Threonine, Valine, or a homologous variant thereof.
  VARIANT 611: note = X288 is selected from Serine, Threonine, Alanine, Valine, or a homologous variant thereof.
  VARIANT 613: note = X289 is selected from Isoleucine, Methionine, Lysine, Valine, Serine, Leucine, Phenylalanine, Arginine, or a homologous variant thereof.
  VARIANT 617: note = X291 is selected from Leucine, Aspartate, Valine, Asparagine, Methionine, Glutamate, Serine, or a homologous variant thereof.
  VARIANT 620: note = X292 is selected from Serine, Asparagine, or a homologous variant thereof.
  VARIANT 621: note = X293 is selected from Alanine, Threonine, Serine, Methionine, or a homologous variant thereof.
  VARIANT 626: note = X294 is selected from Lysine, Glutamine, or a homologous variant thereof.
  VARIANT 628: note = X295 is selected from Leucine, Isoleucine, Serine, or a homologous variant thereof.
  VARIANT 633: note = X298 is selected from Asparagine, Aspartate, Serine, or a homologous variant thereof.
  VARIANT 642: note = X303 is selected from Glutamate, Lysine, or a homologous variant thereof.
  VARIANT 647: note = X304 is selected from Lysine, Arginine, Serine, or a homologous variant thereof.
  VARIANT 649: note = X305 is selected from Arginine, Glutamine, Lysine, Proline, or a homologous variant thereof.
  VARIANT 652: note = X307 is selected from Aspartate, Glycine, Asparagine, Serine, Arginine, or a homologous variant thereof.
  VARIANT 654: note = X308 is selected from Asparagine, Glycine, Glutamate, Aspartate, Valine, or a homologous variant thereof.
  VARIANT 655: note = X309 is selected from Leucine, Asparagine, or a homologous variant thereof.
  VARIANT 657: note = X310 is absent or present and when present is a peptide sequence Insert X310 or a homologous variant thereof.
  VARIANT 659: note = X311 is selected from Tyrosine, Threonine, Leucine, Glutamate, Alanine, Isoleucine, Valine, or a homologous variant thereof.
  VARIANT 660: note = X312 is selected from Aspartate, Glycine, or a homologous variant thereof.
  VARIANT 661: note = X313 is selected from Asparagine, Threonine, Serine, Alanine, Isoleucine, or a homologous variant thereof.
  VARIANT 662: note = X314 is selected from Isoleucine, Asparagine, Lysine, Valine, Threonine, Serine, Aspartate, Alanine, or a homologous variant thereof.
  VARIANT 663: note = X315 is selected from Serine, Glycine, Asparagine, Histidine, Arginine, Alanine, or a homologous variant thereof.
  VARIANT 664: note = X316 is selected from Alanine, Isoleucine, Threonine, Phenylalanine, Serine, Valine, Glutamine, Lysine, or a homologous variant thereof.
  VARIANT 665: note = X317 is selected from Serine, Asparagine, Histidine, Arginine, Alanine, Glycine, or a homologous variant thereof.
  VARIANT 666: note = X318 is selected from Asparagine, Glycine, Alanine, Methionine, Aspartate, Glutamate, or a homologous variant thereof.
  VARIANT 667: note = X319 is selected from Threonine, Valine, Alanine, Leucine, Isoleucine, or a homologous variant thereof.
  VARIANT 669: note = X321 is selected from Leucine, Isoleucine, Proline, Glutamine, or a homologous variant thereof.
  VARIANT 670: note = X322 is selected from Glutamine, Glutamate, Methionine, Isoleucine, Leucine, or a homologous variant thereof.
  VARIANT 672: note = X323 is selected from Glutamine, Serine, Glutamate, or a homologous variant thereof.
  VARIANT 688: note = X329 is selected from Threonine, Isoleucine, or a homologous variant thereof.
  VARIANT 693: note = X331 is absent or present and when present is a peptide sequence Insert X331 or a homologous variant thereof.
  VARIANT 694: note = X332 is selected from Asparagine, Lysine, Aspartate, or a homologous variant thereof.
  VARIANT 695: note = X333 is selected from Threonine, Glutamate, Leucine, Isoleucine, or a homologous variant thereof.
  VARIANT 696: note = X334 is selected from Aspartate, Asparagine, or a homologous variant thereof.
  VARIANT 700: note = X335 is selected from Alanine, Valine, Threonine, Glutamine, or a homologous variant thereof.
  VARIANT 702: note = X336 is selected from Glycine, Tryptophan, or a homologous variant thereof.
  VARIANT 703: note = X337 is selected from Methionine, Threonine, Isoleucine, Lysine, Arginine, or a homologous variant thereof.
  VARIANT 340: note = X340 is selected from Serine, Alanine, Aspartate, Glycine, Asparagine, or a homologous variant thereof.
  VARIANT 715: note = X361 is selected from Serine, Alanine, Valine, Phenylalanine, Threonine, or a homologous variant thereof.
  VARIANT 716: note = X362 is selected from Threonine, Alanine, Tyrosine, or a homologous variant thereof.
  VARIANT 717: note = X363 is selected from Proline, Threonine, Leucine, Alanine, or a homologous variant thereof.
  VARIANT 718: note = X364 is selected from Threonine, Alanine, Serine, Proline, Asparagine, or a homologous variant thereof.
  VARIANT 719: note = X365 is selected from Glutamate, Aspartate, Threonine, Serine, Asparagine, or a homologous variant thereof.
  VARIANT 720: note = X366 is selected from Asparagine, Lysine, Serine, Aspartate, Proline, Glutamate, or a homologous variant thereof.
  VARIANT 721: note = X367 is selected from Glycine, Glutamate, Serine, Proline, Threonine, Asparagine, Aspartate, or a homologous variant thereof.
  VARIANT 722: note = X368 is selected from Glycine, Aspartate, Threonine, Serine, Valine, or a homologous variant thereof.
  VARIANT 723: note = X369 is selected from Asparagine, Aspartate, Serine, or a homologous variant thereof.
  VARIANT 726: note = X372 is selected from Asparagine, Aspartate, Lysine, Threonine, Serine, or a homologous variant thereof.
  VARIANT 729: note = X375 is selected from Threonine, Lysine, Glutamate, Asparagine, Tyrosine, or a homologous variant thereof.
  VARIANT 731: note = X377 is selected from Threonine, Alanine, Serine, Lysine, Proline, or a homologous variant thereof.
  VARIANT 732: note = X378 is selected from Threonine, Glutamate, Alanine, Proline, Serine, Isoleucine, Lysine, or a homologous variant thereof
  VARIANT 765: note = X379 is absent or present and when present is a peptide sequence Insert X379 or a homologous variant thereof.
XAFFXTVIIPAIVGGIATGXXVGTVSGLLSWGLKXAEXANKXPDXPXKVXXIQAGXGFXXFXXKXYDLYXSLLSSKIXGGWDXGNAARHYWVKXGQWNKLEVXMXXAVGTYXLSGLXNFTGGDLDXNMQKATLRLGQFNGNSFTSYKDXXXRTTRVXFXAKNIXIDNFVEINNRVGSGAGRKASSTVLTLXXSXXIXSXXNAEISLYDGATLNLAXSXSVXLXGXVWMGRLQYVGAYLAPSYSTIXTSKVXGEXNFXHLXVGXXNXAQAGIIAXXKTXIGXLDLWQSXGLXIIXPPXGGKXTVVNIXXINTXXDGTIRVGGYKASLTTNAAXLXIGXGGVNLSNXXSGRXLLVENLTGXITVXGXLRVNNQXGGXXLAGSSXNFEFKAGXXTKNXTATFNNXIHLGRXVNLXVDAXTXXHFKXIDXXSDGGFNXXLDFSGVTXKVXINKLTTXATNVXVKNFDIKELIVTTRVQSVGQYTIFXXXIGDXSXIXXVSLQXGYSPIFXGGVTFKXGKKLVIDEFYHAPWNYFDARXITDVEIXKKFLFGAPGXIXGKTGLMFNNLXLXXNAXMDYGKDLDLTIXXXFTNNXXXMNLLVQXXRVAXLNVXXXAXMXFNNXIDXXTGFYXPXIKINXAQNLTKNKXHVLLXAXNIXYXXVXSXXXXXXXXXNXXEXFKERLALYNNNNRMDXCVVRXXXXDIKXCXXAIGNQXMVNNPXXYXYLXGKAWKNXXIXKXAXXSXIXVXXXXNXXXXXXXXXTTXLPXNXXX

SEQ ID NO: 3 - protein, 12 aa, synthetic construct
  VARIANT 2: note = Xp32 is absent or present and when present is Threonine or a homologous variant thereof.
  VARIANT 3: note = Xp33 is absent or present, and when present is selected from Proline and Alanine or homologous variants thereof.
  VARIANT 5: note = Xp35 is present or absent, and when present is selected from Aspartate or Glutamate or homologous variants thereof.
  VARIANT 8: note = Xp38 is absent or present, and when present is selected from Histidine and Arginine or homologous variants thereof
  VARIANT 11: note = Xp311 is present or absent, and when present is selected from Serine or Asparagine, or homologous variants thereof
NXXNXPIXSEXR

SEQ ID NO: 4-5 - skipped (2 entries)

SEQ ID NO: 6 - protein, 21 aa, synthetic construct
  VARIANT 1: note = Xp61 is selected from Alanine, Threonine, or homologous variants thereof
  VARIANT 2: note = Xp62 is selected from Asparagine, Lysine, Tyrosine, or homologous variants thereof
  VARIANT 8: note = Xp68 is selected from Tyrosine, Asparagine, or homologous variants thereof
  VARIANT 19: note = Xp619 is selected from Glycine, Alanine, or homologous variants thereof.
  VARIANT 20: note = Xp620 is selected from Histidine, Asparagine, or homologous variants thereof an
  VARIANT 21: note = Xp621 is selected from Serine, Threonine, or homologous variants thereof
XXFNGNIXLGKSTNLRVNXXX

SEQ ID NO: 7-9 - skipped (3 entries)

SEQ ID NO: 10 - protein, 765 aa, synthetic construct
  VARIANT 1: note = X1 is absent
  VARIANT 218: note = X78 is absent
  VARIANT 297: note = X117 is absent
  VARIANT 418: note = X173 is absent
  VARIANT 427: note = X182 is absent
  VARIANT 434: note = X187 is absent
  VARIANT 657: note = X310 is absent
  VARIANT 657: note = X331 is absent
  VARIANT 765: note = X379 is a peptide sequence Insert X379 or a homologous variant thereof.
XAFFTTVIIPAIVGGIATGTAVGTVSGLLGWGLKQAEEANKTPDKPDKVWRIQAGKGFNEFPNKEYDLYKSLLSSKIDGGWDWGNAATHYWIKGGQWNKLEVDMKDAVGTYKLSGLRNFTGGDLDVNMQKATLRLGQFNGNSFTSYKDSADRTTRVDFNAKNILIDNFLEINNRVGSGAGRKASSTVLTLQASEGITSSKNAEISLYDGATLNLASNXSVKLNGNVWMGRLQYVGAYLAPSYSTINTSKVTGEVNFNHLTVGDHNAAQAGIIASNKTHIGTLDLWQSAGLNIIAPPXGGKDTVVNIDRINTKADGTIKVGGFKASLTTNAAHLNIGKGGVNLSNQASGRTLLVENLTGNITVDGPLRVNNQVGGYALAGSSANFEFKAGVDTKNGTATFNNDISLGRFVNLKVDAHTXANFKGIDTXGNGGFNXTLDFSGVTNKVNINKLITASTNVAVKNFNINELIVKTNGVSVGEYTHFSEDIGSQSRINTVRLETGTRSIFSGGVKFKSGEKLVIDEFYYSPWNYFDARNIKNVEITRKFASSTPENPWGTSKLMFNNLTLGQNAVMDYSQFSNLTIQGDFINNQGTINYLVRGGKVATLNVGNAAAMMFNNDIDSATGFYKPLIKINSAQDLIKNTEHVLLKAKIIGYGNVXSTGTNGISNVNLEEQFKERLALYNNNNRMDTCVVRXNTDDIKACGMAIGNQSMVNNPDNYKYLIGKAWKNIGISKTANGSKISVYYLGNSTPTENGGNTTNLPTNTTX

SEQ ID NO: 11 - protein, 765 aa, synthetic construct
  VARIANT 1: note = X1 is absent
  VARIANT 218: note = X78 is absent
  VARIANT 297: note = X117 is absent
  VARIANT 418: note = X173 is absent
  VARIANT 427: note = X182 is absent
  VARIANT 434: note = X187 is absent
  VARIANT 657: note = X310 is absent
  VARIANT 693: note = X331 is absent
  VARIANT 765: note = X379 is a peptide sequence Insert X379 or a homologous variant thereof.
XAFFTTVIIPAIVGAIATATAVGTVSGLLGWGLKQAEEANKTPDKPDKVWRIQAGKGFNEFPNKEYDLYKSLLSSKIDGGWDWGNAATHYWIKGGQWNKLEVDMKDAVGTYKLSGLRNFTGGDLDVNMQKATLRLGQFNGNSFTSYKDSADRTTRVDFNAKNILIDNFLEINNRVGSGAGRKASSTVLTLQASEGITSSKNAEISLYDGATLNLASNXSVKLNGNVWMGRLQYVGAYLAPSYSTINTSKVTGEVNFNHLTVGDHNAAQAGIIASNKTHIGTLDLWQSAGLNIIAPPXGGKDTVVNIDRINTKADGTIKVGGFKASLTTNAAHLNIGKGGVNLSNQASGRTLLVENLTGNITVDGPLRVNNQVGGYALAGSSANFEFKAGVDTKNGTATFNNDISLGRFVNLKVDAHTXANFKGIDTXGNGGFNXTLDFSGVTNKVNINKLITASTNVAVKNFNINELIVKTNGVSVGEYTHFSEDIGSQSRINTVRLETGTRSIFSGGVKFKSGEKLVIDEFYYSPWNYFDARNIKNVEITRKFASSTPENPWGTSKLMFNNLTLGQNAVMDYSQFSNLTIQGDFINNQGTINYLVRGGKVATLNVGNAAAMMFNNDIDSATGFYKPLIKINSAQDLIKNTEHVLLKAKIIGYGNVXSTGTNGISNVNLEEQFKERLALYNNNNRMDTCVVRXNTDDIKACGMAIGNQSMVNNPDNYKYLIGKAWKNIGISKTANGSKISVYYLGNSTPTENGGNTTNLPTNTTX

SEQ ID NO: 12 - protein, 765 aa, synthetic construct; identical to SEQ ID NO: 10
  VARIANT 1: note = X1 is absent
  VARIANT 218: note = X78 is absent
  VARIANT 297: note = X117 is absent
  VARIANT 418: note = X173 is absent
  VARIANT 427: note = X182 is absent
  VARIANT 434: note = X187 is absent
  VARIANT 657: note = X310 is absent
  VARIANT 693: note = X331 is absent
  VARIANT 765: note = X379 is absent

SEQ ID NO: 13 - protein, 765 aa, synthetic construct; identical to SEQ ID NO: 11
  VARIANT 1: note = X1 is absent
  VARIANT 218: note = X78 is absent
  VARIANT 297: note = X1 17 is absent
  VARIANT 418: note = X173 is absent
  VARIANT 427: note = X182 is absent
  VARIANT 434: note = X187 is absent
  VARIANT 657: note = X310 is absent
  VARIANT 693: note = X331 is absent
  VARIANT 765: note = X379 is absent

SEQ ID NO: 14 - protein, 765 aa, synthetic construct
  VARIANT 1: note = X1 is a peptide sequence of SEQ ID No: 3 or a homologous variant thereof.
  VARIANT 218: note = X78 is a peptide sequence Insert X78 or a homologous variant thereof.
  VARIANT 297: note = X117 is absent
  VARIANT 418: note = X173 is a peptide sequence of SEQ ID NO: 6 or a homologous variant thereof.
  VARIANT 427: note = X182 is a peptide sequence of Insert X182 or a homologous variant thereof.
  VARIANT 434: note = X187 is a peptide sequence Insert X187 or a homologous variant thereof.
  VARIANT 657: note = X310 is a peptide sequence of Insert X310 or a homologous variant thereof.
  VARIANT 693: note = X331 is a peptide sequence Insert X331 or a homologous variant thereof.
  VARIANT 765: note = X379 is a peptide sequence Insert X379 or a homologous variant thereof.
XAFFTTVIIPAIVGAIATAAAVGTVSGLLSWGLKQAEQANKAPDKPDKVWRIQAGRGFDNFPHKQYDLYKSLLSSKIDGGWDWGNAARHYWVKDGQWNKLEVDMQNAVGTYNLSGLINFTGGDLDVNMQKATLRLGQFNGNSFTSFKDGANRTTRVNFDAKNILIDNFVEINNRVGSGAGRKASSTVLTLKSSEKITSRENAEISLYDGATLNLVSSXSVDLYGKVWMGRLQYVGAYLAPSYSTIDTSKVQGEMNFRHLAVGDQNAAQAGIIANKKTNIGTLDLWQSAGLSIITPPXGGKDTVVNIFHLNTKADGTLRAGGFKASLSTNAAHLHIGEGGVNLSNQASGRTLLVENLTGNITVEGTLRVNNQVGGAAIAGSSANFEFKAGEDTNNATATFNNDIHLGKAVNLRVDAHTXAHFKNIDAXSDNGLNXTLDFSGVTDKVNINKLTTAATNVNIKNFDIKELVVTTRVQSFGQYTIFGENIGDKSRIGVVSLQTGYSPAYSGGVTFKGGKKLVIDEIYHAPWNYFDARNVTDVEINKRILFGAPGNIAGKTGLMFNNLTLNSNASMDYGKDLDLTIQGHFTNNQGTMNLFVQDGRVATLNAGHQASMIFNNLVDSTTGFYKPLIKINNAQNLTKNKEHVLVKARNIDYNLVXSYDNISASNTNLQEQFKERLALYNNNNRMDTCVVRXNLNDIKACGMAIGNQSMVNNPENYKYLEGKAWKNTGINKTANNTTIAVNLGNNSTPTNSTTDTTNLPTNTTX

SEQ ID NO: 15 - protein, 765 aa, synthetic construct
  VARIANT 1: note = X1 is a peptide sequence of SEQ ID No: 3 or a homologous variant thereof
  VARIANT 218: note = X78 is a peptide sequence Insert X78 or a homologous variant thereof.
  VARIANT 297: note = X117 is absent
  VARIANT 418: note = X173 is absent
  VARIANT 427: note = X182 is a peptide sequence Insert X182 or a homologous variant thereof.
  VARIANT 434: note = X187 is a peptide sequence of Insert X187 or a homologous variant thereof.
  VARIANT 657: note = X310 is a peptide sequence Insert X310 or a homologous variant thereof.
  VARIANT 693: note = X331 is a peptide sequence Insert X331 or a homologous variant thereof.
  VARIANT 765: note = X379 is a peptide sequence Insert X379 or a homologous variant thereof.
XAFFTTVIIPAIVGGIATGAAVGTVSGLLSWGLKQAEQANKAPDKPDKVWRIQAGRGFDNFPHKQYDLYKSLLSSKIDGGWDWGNAARHYWVKDGQWNKLEVDMQNAVGTYNLSGLINFTGGDLDVNMQKATLRLGQFNGNSFTSFKDGANRTTRVNFDAKNILIDNFVEINNRVGSGAGRKASSTVLTLKSSEKITSRENAEISLYDGATLNLVSSXSVDLYGKVWMGRLQYVGAYLAPSYSTIDTSKVQGEMNFRHLAVGDQNAAQAGIIANKKTNIGTLDLWQSAGLSIITPPXGGKDTVVNIFHLNTKADGTLRAGGFKASLSTNAAHLHIGEGGVNLSNQASGRTLLVENLTGNITVEGTLRVNNQVGGAAIAGSSANFEFKAGEDTNNATATFNNDIHLGKAVNLRVDAHTXAHFKNIDAXSDNGLNXTLDFSGVTDKVNINKLTTAATNVNIKNFDIKELVVTTRVQSFGQYTIFGENIGDKSRIGVVSLQTGYSPAYSGGVTFKGGKKLVIDEIYHAPWNYFDARNVTDVEINKRILFGAPGNIAGKTGLMFNNLTLNSNASMDYGKDLDLTIQGHFTNNQGTMNLFVQDGRVATLNAGHQASMIFNNLVDSTTGFYKPLIKINNAQNLTKNKEHVLVKARNIDYNLVXSYDNISASNTNLQEQFKERLALYNNNNRMDTCVVRXNLNDIKACGMAIGNQSMVNNPENYKYLEGKAWKNTGINKTANNTTIAVNLGNNSTPTNSTTDTTNLPTNTTX

SEQ ID NO: 16 - protein, 765 aa, synthetic construct; identical to SEQ ID NO: 15
  VARIANT 1: note = X1 is a peptide sequence of SEQ ID No: 3 or a homologous variant thereof
  VARIANT 218: note = X78 is is a peptide sequence Insert X78 or a homologous variant thereof.
  VARIANT 297: note = X117 is absent
  VARIANT 418: note = X173 is a peptide sequence of SEQ ID No: 6 or a homologous variant thereof
  VARIANT 427: note = X182 is a peptide sequence Insert X182 or a homologous variant thereof.
  VARIANT 434: note = X187 is a peptide sequence of Insert X187 or a homologous variant thereof.
  VARIANT 657: note = X310 is a peptide sequence Insert X310 or a homologous variant thereof.
  VARIANT 693: note = X331 is a peptide sequence Insert X331 or a homologous variant thereof.
  VARIANT 765: note = X379 is a peptide sequence of Insert X379 or a homologous variant thereof

SEQ ID NO: 17 - protein, 765 aa, synthetic construct; identical to SEQ ID NO: 15
  VARIANT 1: note = X1 is a peptide sequence of SEQ ID No: 3 or a homologous variant thereof
  VARIANT 218: note = X78 is a peptide sequence of Insert X78 or a homologous variant thereof.
  VARIANT 297: note = X117 is absent
  VARIANT 418: note = X173 is absent
  VARIANT 427: note = X182 is a peptide sequence Insert X182 or a homologous variant thereof.
  VARIANT 434: note = X187 is a peptide sequence Insert X187 or a homologous variant thereof.
  VARIANT 657: note = X310 is a peptide sequence Insert X310 or a homologous variant thereof.
  VARIANT 693: note = X331 is a peptide sequence of Insert X331 or a homologous variant thereof.
  VARIANT 765: note = X379 is a peptide sequence Insert X379 or a homologous variant thereof.

SEQ ID NO: 18 - skipped

SEQ ID NO: 19 - protein, 765 aa, synthetic construct; identical to SEQ ID NO: 15
  VARIANT 1: note = X1 is a peptide sequence of SEQ ID No: 3 or a homologous variant thereof
  VARIANT 218: note = X78 is a peptide sequence Insert X78 or a homologous variant thereof.
  VARIANT 297: note = X117 is absent
  VARIANT 418: note = X173 is absent
  VARIANT 427: note = X182 is peptide sequence Insert X182 or a homologous variant thereof.
  VARIANT 434: note = X187 is a peptide sequence Insert X187 or a homologous variant thereof.
  VARIANT 657: note = X310 is a peptide sequence Insert X310 or a homologous variant thereof.
  VARIANT 693: note = X331 is a peptide sequence Insert X331 or a homologous variant thereof.
  VARIANT 765: note = X379 is absent

SEQ ID NO: 20 - protein, 12 aa, synthetic construct
NTPNDPIHSESR

SEQ ID NO: 21-22 - skipped (2 entries)

SEQ ID NO: 23 - protein, 21 aa, synthetic construct
AYFNGNIYLGKSTNLRVNGHS

SEQ ID NO: 24 - protein, 5 aa, synthetic construct
GVQGA

SEQ ID NO: 25 - protein, 9 aa, synthetic construct
NNARFASYA

SEQ ID NO: 26 - protein, 821 aa, synthetic construct
AFFTTVIIPAIVGGIATGTAVGTVSGLLSWGLKQAEEANKTPDKPDKVWRIQAGKGFNEFPNKEYDLYKSLLSSKIDGGWDWGNAARHYWVKGGQWNKLEVDMKDAVGTYKLSGLRNFTGGDLDVNMQKATLRLGQFNGNSFTSYKDSADRTTRVDFNAKNISIDNFVEINNRVGSGAGRKASSTVLTLQASEGITSSKNAEISLYDGATLNLASNSVKLMGNVWMGRLQYVGAYLAPSYSTINTSKVTGEVNFNHLTVGDKNAAQAGIIASNKTHIGTLDLWQSAGLNIIAPPEGGYKDKPNNTPSQSGAKNDKNESAKNNSNTQVINPPNSTQKTEIQPTQVIDGPFAGGKDTVVNINRINTNADGTIRVGGYKASLTTNAAHLNIGKGGVNLSNQASGRSLLVENLTGNITVDGPLRVNNQVGGYALAGSSANFEFKAGVDTKNGTATFNNDISLGRFVNLKVDAHTANFKGIDTGNGGFNTLDFSGVTNKVNINKLITASTNVAVKNFNINELIVKTNGISVGEYTHFSEDIGSQSRINTVRLETGTRSIFSGGVKFKGGEKLVIDEFYYSPWNYFDARNIKNVEITRKFASSTPENPWGTSKLMFNNLTLGQNAVMDYSQFSNLTIQGDFINNQGTINYLVRGGKVATLNVGNAAAMMFNNDIDSATGFYKPLIKINSAQDLIKNTEHVLLKAKIIGYGNVSTGTNSISNVNLEEQFKERLALYNNNNRMDTCVVRNTDDIKACGMAIGNQSMVNNPDNYKYLIGKAWKNIGISKTANGSKISVYYLGNSTPTENGGNTTNLPTNTTNNARFARYA

SEQ ID NO: 27 - skipped

SEQ ID NO: 28 - protein, 821 aa, synthetic construct
AFFTTVIIPAIVGAIATATAVGTVSGLLGWGLKQAEEANKTPDKPDKVWRIQAGKGFNEFPNKEYDLYKSLLSSKIDGGWDWGNAATHYWIKGGQWNKLEVDMKDAVGTYKLSGLRNFTGGDLDVNMQKATLRLGQFNGNSFTSYKDSADRTTRVDFNAKNILIDNFLEINNRVGSGAGRKASSTVLTLQASEGITSSKNAEISLYDGATLNLASNSVKLNGNVWMGRLQYVGAYLAPSYSTINTSKVTGEVNFNHLTVGDHNAAQAGIIASNKTHIGTLDLWQSAGLNIIAPPEGGYKDKPNNTPSQSGAKNDKQESSQNNSNTQVINPPNSTQKTEVQPTQVIDGPFAGGKDTVVNIDRINTKADGTIKVGGFKASLTTNAAHLNIGKGGVNLSNQASGRTLLVENLTGNITVDGPLRVNNQVGGYALAGSSANFEFKAGVDTKNGTATFNNDISLGRFVNLKVDAHTANFKGIDTGNGGFNTLDFSGVTNKVNINKLITASTNVAVKNFNINELIVKTNGVSVGEYTHFSEDIGSQSRINTVRLETGTRSIFSGGVKFKSGEKLVIDEFYYSPWNYFDARNIKNVEITRKFASSTPENPWGTSKLMFNNLTLGQNAVMDYSQFSNLTIQGDFINNQGTINYLVRGGKVATLNVGNAAAMMFNNDIDSATGFYKPLIKINSAQDLIKNTEHVLLKAKIIGYGNVSTGTNGISNVNLEEQFKERLALYNNNNRMDTCVVRNTDDIKACGMAIGNQSMVNNPDNYKYLIGKAWKNIGISKTANGSKISVYYLGNSTPTENGGNTTNLPTNTTNNARFASYA

SEQ ID NO: 29 - skipped

SEQ ID NO: 30 - protein, 812 aa, synthetic construct
AFFTTVIIPAIVGGIATGTAVGTVSGLLGWGLKQAEEANKTPDKPDKVWRIQAGKGFNEFPNKEYDLYKSLLSSKIDGGWDWGNAATHYWIKGGQWNKLEVDMKDAVGTYKLSGLRNFTGGDLDVNMQKATLRLGQFNGNSFTSYKDSADRTTRVDFNAKNILIDNFLEINNRVGSGAGRKASSTVLTLQASEGITSSKNAEISLYDGATLNLASNSVKLNGNVWMGRLQYVGAYLAPSYSTINTSKVTGEVNFNHLTVGDHNAAQAGIIASNKTHIGTLDLWQSAGLNIIAPPEGGYKDKPNNTPSQSGAKNDKQESSQNNSNTQVINPPNSTQKTEVQPTQVIDGPFAGGKDTVVNIDRINTKADGTIKVGGFKASLTTNAAHLNIGKGGVNLSNQASGRTLLVENLTGNITVDGPLRVNNQVGGYALAGSSANFEFKAGVDTKNGTATFNNDISLGRFVNLKVDAHTANFKGIDTGNGGFNTLDFSGVTNKVNINKLITASTNVAVKNFNINELIVKTNGVSVGEYTHFSEDIGSQSRINTVRLETGTRSIFSGGVKFKSGEKLVIDEFYYSPWNYFDARNIKNVEITRKFASSTPENPWGTSKLMFNNLTLGQNAVMDYSQFSNLTIQGDFINNQGTINYLVRGGKVATLNVGNAAAMMFNNDIDSATGFYKPLIKINSAQDLIKNTEHVLLKAKIIGYGNVSTGTNGISNVNLEEQFKERLALYNNNNRMDTCVVRNTDDIKACGMAIGNQSMVNNPDNYKYLIGKAWKNIGISKTANGSKISVYYLGNSTPTENGGNTTNLPTNTT

SEQ ID NO: 31 - protein, 765 aa, synthetic construct
AFFTTVIIPAIVGGIATGTAVGTVSGLLGWGLKQAEEANKTPDKPDKVWRIQAGKGFNEFPNKEYDLYKSLLSSKIDGGWDWGNAATHYWIKGGQWNKLEVDMKDAVGTYKLSGLRNFTGGDLDVNMQKATLRLGQFNGNSFTSYKDSADRTTRVDFNAKNILIDNFLEINNRVGSGAGRKASSTVLTLQASEGITSSKNAEISLYDGATLNLASNSVKLNGNVWMGRLQYVGAYLAPSYSTINTSKVTGEVNFNHLTVGDHNAAQAGIIASNKTHIGTLDLWQSAGLNIIAPPGGKDTVVNIDRINTKADGTIKVGGFKASLTTNAAHLNIGKGGVNLSNQASGRTLLVENLTGNITVDGPLRVNNQVGGYALAGSSANFEFKAGVDTKNGTATFNNDISLGRFVNLKVDAHTANFKGIDTGNGGFNTLDFSGVTNKVNINKLITASTNVAVKNFNINELIVKTNGVSVGEYTHFSEDIGSQSRINTVRLETGTRSIFSGGVKFKSGEKLVIDEFYYSPWNYFDARNIKNVEITRKFASSTPENPWGTSKLMFNNLTLGQNAVMDYSQFSNLTIQGDFINNQGTINYLVRGGKVATLNVGNAAAMMFNNDIDSATGFYKPLIKINSAQDLIKNTEHVLLKAKIIGYGNVSTGTNGISNVNLEEQFKERLALYNNNNRMDTCVVRNTDDIKACGMAIGNQSMVNNPDNYKYLIGKAWKNIGISKTANGSKISVYYLGNSTPTENGGNTTNLPTNTTNNARFASYA

SEQ ID NO: 32 - protein, 765 aa, synthetic construct
AFFTTVIIPAIVGAIATATAVGTVSGLLGWGLKQAEEANKTPDKPDKVWRIQAGKGFNEFPNKEYDLYKSLLSSKIDGGWDWGNAATHYWIKGGQWNKLEVDMKDAVGTYKLSGLRNFTGGDLDVNMQKATLRLGQFNGNSFTSYKDSADRTTRVDFNAKNILIDNFLEINNRVGSGAGRKASSTVLTLQASEGITSSKNAEISLYDGATLNLASNSVKLNGNVWMGRLQYVGAYLAPSYSTINTSKVTGEVNFNHLTVGDHNAAQAGIIASNKTHIGTLDLWQSAGLNIIAPPGGKDTVVNIDRINTKADGTIKVGGFKASLTTNAAHLNIGKGGVNLSNQASGRTLLVENLTGNITVDGPLRVNNQVGGYALAGSSANFEFKAGVDTKNGTATFNNDISLGRFVNLKVDAHTANFKGIDTGNGGFNTLDFSGVTNKVNINKLITASTNVAVKNFNINELIVKTNGVSVGEYTHFSEDIGSQSRINTVRLETGTRSIFSGGVKFKSGEKLVIDEFYYSPWNYFDARNIKNVEITRKFASSTPENPWGTSKLMFNNLTLGQNAVMDYSQFSNLTIQGDFINNQGTINYLVRGGKVATLNVGNAAAMMFNNDIDSATGFYKPLIKINSAQDLIKNTEHVLLKAKIIGYGNVSTGTNGISNVNLEEQFKERLALYNNNNRMDTCVVRNTDDIKACGMAIGNQSMVNNPDNYKYLIGKAWKNIGISKTANGSKISVYYLGNSTPTENGGNTTNLPTNTTNNARFASYA

SEQ ID NO: 33 - protein, 756 aa, synthetic construct
AFFTTVIIPAIVGGIATGTAVGTVSGLLGWGLKQAEEANKTPDKPDKVWRIQAGKGFNEFPNKEYDLYKSLLSSKIDGGWDWGNAATHYWIKGGQWNKLEVDMKDAVGTYKLSGLRNFTGGDLDVNMQKATLRLGQFNGNSFTSYKDSADRTTRVDFNAKNILIDNFLEINNRVGSGAGRKASSTVLTLQASEGITSSKNAEISLYDGATLNLASNSVKLNGNVWMGRLQYVGAYLAPSYSTINTSKVTGEVNFNHLTVGDHNAAQAGIIASNKTHIGTLDLWQSAGLNIIAPPGGKDTVVNIDRINTKADGTIKVGGFKASLTTNAAHLNIGKGGVNLSNQASGRTLLVENLTGNITVDGPLRVNNQVGGYALAGSSANFEFKAGVDTKNGTATFNNDISLGRFVNLKVDAHTANFKGIDTGNGGFNTLDFSGVTNKVNINKLITASTNVAVKNFNINELIVKTNGVSVGEYTHFSEDIGSQSRINTVRLETGTRSIFSGGVKFKSGEKLVIDEFYYSPWNYFDARNIKNVEITRKFASSTPENPWGTSKLMFNNLTLGQNAVMDYSQFSNLTIQGDFINNQGTINYLVRGGKVATLNVGNAAAMMFNNDIDSATGFYKPLIKINSAQDLIKNTEHVLLKAKIIGYGNVSTGTNGISNVNLEEQFKERLALYNNNNRMDTCVVRNTDDIKACGMAIGNQSMVNNPDNYKYLIGKAWKNIGISKTANGSKISVYYLGNSTPTENGGNTTNLPTNTT

SEQ ID NO: 34 - protein, 756 aa, synthetic construct
AFFTTVIIPAIVGAIATATAVGTVSGLLGWGLKQAEEANKTPDKPDKVWRIQAGKGFNEFPNKEYDLYKSLLSSKIDGGWDWGNAATHYWIKGGQWNKLEVDMKDAVGTYKLSGLRNFTGGDLDVNMQKATLRLGQFNGNSFTSYKDSADRTTRVDFNAKNILIDNFLEINNRVGSGAGRKASSTVLTLQASEGITSSKNAEISLYDGATLNLASNSVKLNGNVWMGRLQYVGAYLAPSYSTINTSKVTGEVNFNHLTVGDHNAAQAGIIASNKTHIGTLDLWQSAGLNIIAPPGGKDTVVNIDRINTKADGTIKVGGFKASLTTNAAHLNIGKGGVNLSNQASGRTLLVENLTGNITVDGPLRVNNQVGGYALAGSSANFEFKAGVDTKNGTATFNNDISLGRFVNLKVDAHTANFKGIDTGNGGFNTLDFSGVTNKVNINKLITASTNVAVKNFNINELIVKTNGVSVGEYTHFSEDIGSQSRINTVRLETGTRSIFSGGVKFKSGEKLVIDEFYYSPWNYFDARNIKNVEITRKFASSTPENPWGTSKLMFNNLTLGQNAVMDYSQFSNLTIQGDFINNQGTINYLVRGGKVATLNVGNAAAMMFNNDIDSATGFYKPLIKINSAQDLIKNTEHVLLKAKIIGYGNVSTGTNGISNVNLEEQFKERLALYNNNNRMDTCVVRNTDDIKACGMAIGNQSMVNNPDNYKYLIGKAWKNIGISKTANGSKISVYYLGNSTPTENGGNTTNLPTNTT

SEQ ID NO: 35-36 - skipped (2 entries)

SEQ ID NO: 37 - protein, 812 aa, synthetic construct
NTPNDPIHSESRAFFTTVIIPAIVGGIATGAAVGTVSGLLSWGLKQAEQANKAPDKPDKVWRIQAGRGFDNFPHKQYDLYKSLLSSKIDGGWDWGNAARHYWVKDGQWNKLEVDMQNAVGTYNLSGLINFTGGDLDVNMQKATLRLGQFNGNSFTSFKDSADRTTRVNFDAKNILIDNFVEINNRVGSGAGRKASSTVLTLKSSEKITSRENAEISLYDGATLNLVSSSNQSVDLYGKVWMGRLQYVGAYLAPSYSTIDTSKVQGEMNFRHLAVGDQNAAQAGIIANKKTNIGTLDLWQSAGLSIITPPGGKDTVVNIFHLNTKADGTLRAGGFKASLSTNAAHLNIGEGGVNLSNQASGRSLLVENLTGNITVEGTLRVNNQVGGAAVAGSSANFEFKAGEDTNNATATFNNDIHLGKAVNLRVDAHTAYFNGNIYLGKSTNLRVNGHSAHFKNIDASKSDNGLNTSALDFSGVTDKVNINKLTTSATNVNIKNFDIKELVVTTRVQSFGQYTIFGENIGDKSRIGVVSLQTGYSPAYSGGVTFKSGKKLVIDEIYHAPWNYFDARNVTDVEINKKILFGAPGNIAGKTGLMFNNLTLNSNASMDYGKDLDLTIQGHFTNNQGTMNLFVQDGRVATLNAGHQASMIFNNLVDSATGFYKPLIKINNAQNLTKNKEHVLVKARNIDYNLVGVQGASYDNISASNTNLQEQFKERLALYNNNNRMDTCVVRKDNLNDIKACGMAIGNQSMVNNPENYKYLEGKAWKNTGINKTANNTTIAVNLGNNSTPTSSESNTTNLPTNTTNNARFARYA

SEQ ID NO: 38 - protein, 791 aa, synthetic construct
NTPNDPIHSESRAFFTTVIIPAIVGGIATGAAVGTVSGLLSWGLKQAEQANKAPDKPDKVWRIQAGRGFDNFPHKQYDLYKSLLSSKIDGGWDWGNAARHYWVKDGQWNKLEVDMQNAVGTYNLSGLINFTGGDLDVNMQKATLRLGQFNGNSFTSFKDSADRTTRVNFDAKNILIDNFVEINNRVGSGAGRKASSTVLTLKSSEKITSRENAEISLYDGATLNLVSSSNQSVDLYGKVWMGRLQYVGAYLAPSYSTIDTSKVQGEMNFRHLAVGDQNAAQAGIIANKKTNIGTLDLWQSAGLSIITPPGGKDTVVNIFHLNTKADGTLRAGGFKASLSTNAAHLNIGEGGVNLSNQASGRSLLVENLTGNITVEGTLRVNNQVGGAAVAGSSANFEFKAGEDTNNATATFNNDIHLGKAVNLRVDAHTAHFKNIDASKSDNGLNTSALDFSGVTDKVNINKLTTSATNVNIKNFDIKELVVTTRVQSFGQYTIFGENIGDKSRIGVVSLQTGYSPAYSGGVTFKSGKKLVIDEIYHAPWNYFDARNVTDVEINKKILFGAPGNIAGKTGLMFNNLTLNSNASMDYGKDLDLTIQGHFTNNQGTMNLFVQDGRVATLNAGHQASMIFNNLVDSATGFYKPLIKINNAQNLTKNKEHVLVKARNIDYNLVGVQGASYDNISASNTNLQEQFKERLALYNNNNRMDTCVVRKDNLNDIKACGMAIGNQSMVNNPENYKYLEGKAWKNTGINKTANNTTIAVNLGNNSTPTSSESNTTNLPTNTTNNARFARYA

SEQ ID NO: 39 - skipped

SEQ ID NO: 40 - protein, 782 aa, synthetic construct
NTPNDPIHSESRAFFTTVIIPAIVGGIATGAAVGTVSGLLSWGLKQAEQANKAPDKPDKVWRIQAGRGFDNFPHKQYDLYKSLLSSKIDGGWDWGNAARHYWVKDGQWNKLEVDMQNAVGTYNLSGLINFTGGDLDVNMQKATLRLGQFNGNSFTSFKDSADRTTRVNFDAKNILIDNFVEINNRVGSGAGRKASSTVLTLKSSEKITSRENAEISLYDGATLNLVSSSNQSVDLYGKVWMGRLQYVGAYLAPSYSTIDTSKVQGEMNFRHLAVGDQNAAQAGIIANKKTNIGTLDLWQSAGLSIITPPGGKDTVVNIFHLNTKADGTLRAGGFKASLSTNAAHLNIGEGGVNLSNQASGRSLLVENLTGNITVEGTLRVNNQVGGAAVAGSSANFEFKAGEDTNNATATFNNDIHLGKAVNLRVDAHTAHFKNIDASKSDNGLNTSALDFSGVTDKVNINKLTTSATNVNIKNFDIKELVVTTRVQSFGQYTIFGENIGDKSRIGVVSLQTGYSPAYSGGVTFKSGKKLVIDEIYHAPWNYFDARNVTDVEINKKILFGAPGNIAGKTGLMFNNLTLNSNASMDYGKDLDLTIQGHFTNNQGTMNLFVQDGRVATLNAGHQASMIFNNLVDSATGFYKPLIKINNAQNLTKNKEHVLVKARNIDYNLVGVQGASYDNISASNTNLQEQFKERLALYNNNNRMDTCVVRKDNLNDIKACGMAIGNQSMVNNPENYKYLEGKAWKNTGINKTANNTTIAVNLGNNSTPTSSESNTTNLPTNTT

SEQ ID NO: 41 - protein, 803 aa, synthetic construct
NTPNDPIHSESRAFFTTVIIPAIVGGIATGAAVGTVSGLLSWGLKQAEQANKAPDKPDKVWRIQAGRGFDNFPHKQYDLYKSLLSSKIDGGWDWGNAARHYWVKDGQWNKLEVDMQNAVGTYNLSGLINFTGGDLDVNMQKATLRLGQFNGNSFTSFKDSADRTTRVNFDAKNILIDNFVEINNRVGSGAGRKASSTVLTLKSSEKITSRENAEISLYDGATLNLVSSSNQSVDLYGKVWMGRLQYVGAYLAPSYSTIDTSKVQGEMNFRHLAVGDQNAAQAGIIANKKTNIGTLDLWQSAGLSIITPPGGKDTVVNIFHLNTKADGTLRAGGFKASLSTNAAHLNIGEGGVNLSNQASGRSLLVENLTGNITVEGTLRVNNQVGGAAVAGSSANFEFKAGEDTNNATATFNNDIHLGKAVNLRVDAHTANFNGNIYLGKSTNLRVNGHTAHFKNIDASKSDNGLNTSALDFSGVTDKVNINKLTTSATNVNIKNFDIKELVVTTRVQSFGQYTIFGENIGDKSRIGVVSLQTGYSPAYSGGVTFKSGKKLVIDEIYHAPWNYFDARNVTDVEINKKILFGAPGNIAGKTGLMFNNLTLNSNASMDYGKDLDLTIQGHFTNNQGTMNLFVQDGRVATLNAGHQASMIFNNLVDSATGFYKPLIKINNAQNLTKNKEHVLVKARNIDYNLVGVQGASYDNISASNTNLQEQFKERLALYNNNNRMDTCVVRKDNLNDIKACGMAIGNQSMVNNPENYKYLEGKAWKNTGINKTANNTTIAVNLGNNSTPTSSESNTTNLPTNTT

SEQ ID NO: 42 - protein, 782 aa, synthetic construct
NTPNDPIHSESRAFFTTVIIPAIVGAIATAAAVGTVSGLLSWGLKQAEQANKAPDKPDKVWRIQAGRGFDNFPHKQYDLYKSLLSSKIDGGWDWGNAARHYWVKDGQWNKLEVDMQNAVGTYNLSGLINFTGGDLDVNMQKATLRLGQFNGNSFTSFKDSADRTTRVNFDAKNILIDNFVEINNRVGSGAGRKASSTVLTLKSSEKITSRENAEISLYDGATLNLVSSSNQSVDLYGKVWMGRLQYVGAYLAPSYSTIDTSKVQGEMNFRHLAVGDQNAAQAGIIANKKTNIGTLDLWQSAGLSIITPPGGKDTVVNIFHLNTKADGTLRAGGFKASLSTNAAHLNIGEGGVNLSNQASGRSLLVENLTGNITVEGTLRVNNQVGGAAVAGSSANFEFKAGEDTNNATATFNNDIHLGKAVNLRVDAHTAHFKNIDASKSDNGLNTSALDFSGVTDKVNINKLTTSATNVNIKNFDIKELVVTTRVQSFGQYTIFGENIGDKSRIGVVSLQTGYSPAYSGGVTFKSGKKLVIDEIYHAPWNYFDARNVTDVEINKKILFGAPGNIAGKTGLMFNNLTLNSNASMDYGKDLDLTIQGHFTNNQGTMNLFVQDGRVATLNAGHQASMIFNNLVDSATGFYKPLIKINNAQNLTKNKEHVLVKARNIDYNLVGVQGASYDNISASNTNLQEQFKERLALYNNNNRMDTCVVRKDNLNDIKACGMAIGNQSMVNNPENYKYLEGKAWKNTGINKTANNTTIAVNLGNNSTPTSSESNTTNLPTNTT

SEQ ID NO: 43 - protein, 803 aa, synthetic construct
NTPNDPIHSESRAFFTTVIIPAIVGAIATAAAVGTVSGLLSWGLKQAEQANKAPDKPDKVWRIQAGRGFDNFPHKQYDLYKSLLSSKIDGGWDWGNAARHYWVKDGQWNKLEVDMQNAVGTYNLSGLINFTGGDLDVNMQKATLRLGQFNGNSFTSFKDSADRTTRVNFDAKNILIDNFVEINNRVGSGAGRKASSTVLTLKSSEKITSRENAEISLYDGATLNLVSSSNQSVDLYGKVWMGRLQYVGAYLAPSYSTIDTSKVQGEMNFRHLAVGDQNAAQAGIIANKKTNIGTLDLWQSAGLSIITPPGGKDTVVNIFHLNTKADGTLRAGGFKASLSTNAAHLNIGEGGVNLSNQASGRSLLVENLTGNITVEGTLRVNNQVGGAAVAGSSANFEFKAGEDTNNATATFNNDIHLGKAVNLRVDAHTANFNGNIYLGKSTNLRVNGHTAHFKNIDASKSDNGLNTSALDFSGVTDKVNINKLTTSATNVNIKNFDIKELVVTTRVQSFGQYTIFGENIGDKSRIGVVSLQTGYSPAYSGGVTFKSGKKLVIDEIYHAPWNYFDARNVTDVEINKKILFGAPGNIAGKTGLMFNNLTLNSNASMDYGKDLDLTIQGHFTNNQGTMNLFVQDGRVATLNAGHQASMIFNNLVDSATGFYKPLIKINNAQNLTKNKEHVLVKARNIDYNLVGVQGASYDNISASNTNLQEQFKERLALYNNNNRMDTCVVRKDNLNDIKACGMAIGNQSMVNNPENYKYLEGKAWKNTGINKTANNTTIAVNLGNNSTPTSSESNTTNLPTNTT